European Patent Application EP 4 180 449 A1, published May 17, 2023. Title: CHIMERIC RECEPTORS AND METHODS OF USE THEREOF. Applicant: KITE PHARMA, INC. Application EP. The sequence listing filed with the application follows.

SEQUENCE LISTING (147 sequences)

SEQ ID NO: 1 - DNA, 294 bp, Homo sapiens
  source 1..294: mol_type = other DNA
cttgataatgaaaagtcaaacggaacaatcattcacgtgaagggcaagcacctctgtccgtcacccttgttccctggtccatccaagccattctgggtgttggtcgtagtgggtggagtcctcgcttgttactctctgctcgtcaccgtggcttttataatcttctgggttagatccaaaagaagccgcctgctccatagcgattacatgaatatgactccacgccgccctggccccacaaggaaacactaccagccttacgcaccacctagagatttcgctgcctatcggagc

SEQ ID NO: 2 - protein, 98 aa, Homo sapiens
LDNEKSNGTIIHVKGKHLCPSPLFPGPSKPFWVLVVVGGVLACYSLLVTVAFIIFWVRSKRSRLLHSDYMNMTPRRPGPTRKHYQPYAPPRDFAAYRS

SEQ ID NO: 3 - DNA, 90 bp, Homo sapiens
  source 1..90: mol_type = other DNA
cttgataatgaaaagtcaaacggaacaatcattcacgtgaagggcaagcacctctgtccgtcacccttgttccctggtccatccaagcca

SEQ ID NO: 4 - protein, 30 aa, Homo sapiens
LDNEKSNGTIIHVKGKHLCPSPLFPGPSKP

SEQ ID NO: 5 - DNA, 81 bp, Homo sapiens
  source 1..81: mol_type = other DNA
ttctgggtgttggtcgtagtgggtggagtcctcgcttgttactctctgctcgtcaccgtggcttttataatcttctgggtt

SEQ ID NO: 6 - protein, 27 aa, Homo sapiens
FWVLVVVGGVLACYSLLVTVAFIIFWV

SEQ ID NO: 7 - DNA, 123 bp, Homo sapiens
  source 1..123: mol_type = other DNA
agatccaaaagaagccgcctgctccatagcgattacatgaatatgactccacgccgccctggccccacaaggaaacactaccagccttacgcaccacctagagatttcgctgcctatcggagc

SEQ ID NO: 8 - protein, 41 aa, Homo sapiens
RSKRSRLLHSDYMNMTPRRPGPTRKHYQPYAPPRDFAAYRS

SEQ ID NO: 9 - DNA, 336 bp, Homo sapiens
  source 1..336: mol_type = other DNA
agggtgaagttttccagatctgcagatgcaccagcgtatcagcagggccagaaccaactgtataacgagctcaacctgggacgcagggaagagtatgacgttttggacaagcgcagaggacgggaccctgagatgggtggcaaaccaagacgaaaaaacccccaggagggtctctataatgagctgcagaaggataagatggctgaagcctattctgaaataggcatgaaaggagagcggagaaggggaaaagggcacgacggtttgtaccagggactcagcactgctacgaaggatacttatgacgctctccacatgcaagccctgccacctagg

SEQ ID NO: 10 - protein, 112 aa, Homo sapiens
RVKFSRSADAPAYQQGQNQLYNELNLGRREEYDVLDKRRGRDPEMGGKPRRKNPQEGLYNELQKDKMAEAYSEIGMKGERRRGKGHDGLYQGLSTATKDTYDALHMQALPPR

SEQ ID NO: 11 - DNA, 117 bp, Homo sapiens
  source 1..117: mol_type = other DNA
attgaggtgatgtatccaccgccttacctggataacgaaaagagtaacggtaccatcattcacgtgaaaggtaaacacctgtgtccttctcccctcttccccgggccatcaaagccc

SEQ ID NO: 12 - protein, 39 aa, Homo sapiens
IEVMYPPPYLDNEKSNGTIIHVKGKHLCPSPLFPGPSKP

SEQ ID NO: 13 - DNA, 288 bp, Homo sapiens
  source 1..288: mol_type = other DNA
gctgcagcattgagcaactcaataatgtattttagtcactttgtaccagtgttcttgccggctaagcctactaccacacccgctccacggccacctaccccagctcctaccatcgcttcacagcctctgtccctgcgcccagaggcttgccgaccggccgcagggggcgctgttcataccagaggactggatttcgcctgcgatatctatatctgggcacccctggccggaacctgcggcgtactcctgctgtccctggtcatcacgctctattgtaatcacaggaac

SEQ ID NO: 14 - protein, 96 aa, Homo sapiens
AAALSNSIMYFSHFVPVFLPAKPTTTPAPRPPTPAPTIASQPLSLRPEACRPAAGGAVHTRGLDFACDIYIWAPLAGTCGVLLLSLVITLYCNHRN

SEQ ID NO: 15 - DNA, 366 bp, synthetic construct
  misc_feature 1..366: note = Description of Artificial Sequence: Syntheticpolynucleotide
  source 1..366: mol_type = other DNA
caggtgcagctgcaggaatccggaccggggctggtgaagcccagcgagactctgagtctcacgtgtacagtttctggaggtagcattagctcctactattggtcatggataaggcagccccccgggaagggattggaatggatcggctatatttactacagtgggagcaccaattacaacccctcactgaagtctagagttacaatcagcgttgacacctcaaagaatcagttcagtttgaaattgtctagcgtcacagcagctgatacagccgtctattattgtgtttctctggtctattgcggtggggattgttacagtggctttgactattgggggcagggtactctggttacagtttcttcc

SEQ ID NO: 16 - protein, 122 aa, synthetic construct
  REGION 1..122: note = Description of Artificial Sequence: Syntheticpolypeptide
QVQLQESGPGLVKPSETLSLTCTVSGGSISSYYWSWIRQPPGKGLEWIGYIYYSGSTNYNPSLKSRVTISVDTSKNQFSLKLSSVTAADTAVYYCVSLVYCGGDCYSGFDYWGQGTLVTVSS

SEQ ID NO: 17 - protein, 7 aa, synthetic construct
  REGION 1..7: note = Description of Artificial Sequence: Syntheticpeptide
GGSISSY

SEQ ID NO: 18 - protein, 5 aa, synthetic construct
  REGION 1..5: note = Description of Artificial Sequence: Syntheticpeptide
YYSGS

SEQ ID NO: 19 - protein, 14 aa, synthetic construct
  REGION 1..14: note = Description of Artificial Sequence: Syntheticpeptide
LVYCGGDCYSGFDY

SEQ ID NO: 20 - DNA, 324 bp, synthetic construct
  misc_feature 1..324: note = Description of Artificial Sequence: Syntheticpolynucleotide
  source 1..324: mol_type = other DNA
gacatccagttgacacagagcccgagttccttgtccgcctccgtcggggatagagtgtcatttacctgtcaggcctctcaggatattaataactttctgaattggtatcagcaaaagcccggaaaggcacccaagctgttgatttacgacgccagtaacctggagacaggcgtgccctcccggtttagtggtagcggaagcggtacggattttacctttactatcagctctctccaacccgaagacattgcaacctactattgtcaacaatatggaaacctgccttttacatttggcggcggcaccaaggtggagattaagcgg

SEQ ID NO: 21 - protein, 108 aa, synthetic construct
  REGION 1..108: note = Description of Artificial Sequence: Syntheticpolypeptide
DIQLTQSPSSLSASVGDRVSFTCQASQDINNFLNWYQQKPGKAPKLLIYDASNLETGVPSRFSGSGSGTDFTFTISSLQPEDIATYYCQQYGNLPFTFGGGTKVEIKR

SEQ ID NO: 22 - protein, 11 aa, synthetic construct
  REGION 1..11: note = Description of Artificial Sequence: Syntheticpeptide
QASQDINNFLN

SEQ ID NO: 23 - protein, 7 aa, synthetic construct
  REGION 1..7: note = Description of Artificial Sequence: Syntheticpeptide
DASNLET

SEQ ID NO: 24 - protein, 9 aa, synthetic construct
  REGION 1..9: note = Description of Artificial Sequence: Syntheticpeptide
QQYGNLPFT

SEQ ID NO: 25 - DNA, 1440 bp, synthetic construct
  misc_feature 1..1440: note = Description of Artificial Sequence: Syntheticpolynucleotide
  source 1..1440: mol_type = other DNA
atggcactccccgtaactgctctgctgctgccgttggcattgctcctgcacgccgcacgcccgcaggtccaactgcaagaaagcggacccggactggtgaagccttctgagacacttagtctgacgtgcacggtcagtggcggctccatctcctcctattattggtcatggatacgacaacccccaggtaagggcctggaatggattggctatatctactattcaggaagcacgaactacaatcccagcctgaagtcccgagtgacaatttcagtagataccagtaaaaaccagttcagtcttaaactgtcaagcgtgacagctgccgacaccgctgtgtattactgcgtctcactggtgtattgtggaggggattgttatagcgggttcgattattggggacagggaaccctggtgactgtatcttccggcggcggcggctcagggggtggcggtagtggcggtgggggttccgatattcaactgacacaatcccccagctcactcagcgccagcgtgggggacagggttagctttacctgtcaagcctctcaggatataaataactttctgaactggtatcaacagaagcctgggaaggcgcccaaactcctgatctatgatgcgtccaacctggaaactggcgtgccttcacgctttagcggctctggcagtggtacagacttcacttttaccatctcttcacttcagccggaggacatcgccacatattactgtcaacagtacggaaacttgccctttacttttggaggcggcaccaaagttgaaatcaaaagggccgctgccctggataacgaaaagagcaatgggactataatacatgttaaaggaaaacacctgtgtccatctcccctgttccctggaccgtcaaagccattttgggtgctcgtggttgtcggtggcgttctcgcctgttatagcttgctggtgacagtagccttcattatcttttgggtgagatccaaaagaagccgcctgctccatagcgattacatgaatatgactccacgccgccctggccccacaaggaaacactaccagccttacgcaccacctagagatttcgctgcctatcggagcagggtgaagttttccagatctgcagatgcaccagcgtatcagcagggccagaaccaactgtataacgagctcaacctgggacgcagggaagagtatgacgttttggacaagcgcagaggacgggaccctgagatgggtggcaaaccaagacgaaaaaacccccaggagggtctctataatgagctgcagaaggataagatggctgaagcctattctgaaataggcatgaaaggagagcggagaaggggaaaagggcacgacggtttgtaccagggactcagcactgctacgaaggatacttatgacgctctccacatgcaagccctgccacctaggtaa

SEQ ID NO: 26 - protein, 479 aa, synthetic construct
  REGION 1..479: note = Description of Artificial Sequence: Syntheticpolypeptide
MALPVTALLLPLALLLHAARPQVQLQESGPGLVKPSETLSLTCTVSGGSISSYYWSWIRQPPGKGLEWIGYIYYSGSTNYNPSLKSRVTISVDTSKNQFSLKLSSVTAADTAVYYCVSLVYCGGDCYSGFDYWGQGTLVTVSSGGGGSGGGGSGGGGSDIQLTQSPSSLSASVGDRVSFTCQASQDINNFLNWYQQKPGKAPKLLIYDASNLETGVPSRFSGSGSGTDFTFTISSLQPEDIATYYCQQYGNLPFTFGGGTKVEIKRAAALDNEKSNGTIIHVKGKHLCPSPLFPGPSKPFWVLVVVGGVLACYSLLVTVAFIIFWVRSKRSRLLHSDYMNMTPRRPGPTRKHYQPYAPPRDFAAYRSRVKFSRSADAPAYQQGQNQLYNELNLGRREEYDVLDKRRGRDPEMGGKPRRKNPQEGLYNELQKDKMAEAYSEIGMKGERRRGKGHDGLYQGLSTATKDTYDALHMQALPPR

SEQ ID NO: 27 - DNA, 1374 bp, synthetic construct
  misc_feature 1..1374: note = Description of Artificial Sequence: Syntheticpolynucleotide
  source 1..1374: mol_type = other DNA
caggtccaactgcaagaaagcggacccggactggtgaagccttctgagacacttagtctgacgtgcacggtcagtggcggctccatctcctcctattattggtcatggatacgacaacccccaggtaagggcctggaatggattggctatatctactattcaggaagcacgaactacaatcccagcctgaagtcccgagtgacaatttcagtagataccagtaaaaaccagttcagtcttaaactgtcaagcgtgacagctgccgacaccgctgtgtattactgcgtctcactggtgtattgtggaggggattgttatagcgggttcgattattggggacagggaaccctggtgactgtatcttccggcggcggcggctcagggggtggcggtagtggcggtgggggttccgatattcaactgacacaatcccccagctcactcagcgccagcgtgggggacagggttagctttacctgtcaagcctctcaggatataaataactttctgaactggtatcaacagaagcctgggaaggcgcccaaactcctgatctatgatgcgtccaacctggaaactggcgtgccttcacgctttagcggctctggcagtggtacagacttcacttttaccatctcttcacttcagccggaggacatcgccacatattactgtcaacagtacggaaacttgccctttacttttggaggcggcaccaaagttgaaatcaaaagggccgctgccctggataacgaaaagagcaatgggactataatacatgttaaaggaaaacacctgtgtccatctcccctgttccctggaccgtcaaagccattttgggtgctcgtggttgtcggtggcgttctcgcctgttatagcttgctggtgacagtagccttcattatcttttgggtgagatccaaaagaagccgcctgctccatagcgattacatgaatatgactccacgccgccctggccccacaaggaaacactaccagccttacgcaccacctagagatttcgctgcctatcggagcagggtgaagttttccagatctgcagatgcaccagcgtatcagcagggccagaaccaactgtataacgagctcaacctgggacgcagggaagagtatgacgttttggacaagcgcagaggacgggaccctgagatgggtggcaaaccaagacgaaaaaacccccaggagggtctctataatgagctgcagaaggataagatggctgaagcctattctgaaataggcatgaaaggagagcggagaaggggaaaagggcacgacggtttgtaccagggactcagcactgctacgaaggatacttatgacgctctccacatgcaagccctgccacctagg

SEQ ID NO: 28 - protein, 458 aa, synthetic construct
  REGION 1..458: note = Description of Artificial Sequence: Syntheticpolypeptide
QVQLQESGPGLVKPSETLSLTCTVSGGSISSYYWSWIRQPPGKGLEWIGYIYYSGSTNYNPSLKSRVTISVDTSKNQFSLKLSSVTAADTAVYYCVSLVYCGGDCYSGFDYWGQGTLVTVSSGGGGSGGGGSGGGGSDIQLTQSPSSLSASVGDRVSFTCQASQDINNFLNWYQQKPGKAPKLLIYDASNLETGVPSRFSGSGSGTDFTFTISSLQPEDIATYYCQQYGNLPFTFGGGTKVEIKRAAALDNEKSNGTIIHVKGKHLCPSPLFPGPSKPFWVLVVVGGVLACYSLLVTVAFIIFWVRSKRSRLLHSDYMNMTPRRPGPTRKHYQPYAPPRDFAAYRSRVKFSRSADAPAYQQGQNQLYNELNLGRREEYDVLDKRRGRDPEMGGKPRRKNPQEGLYNELQKDKMAEAYSEIGMKGERRRGKGHDGLYQGLSTATKDTYDALHMQALPPR

SEQ ID NO: 29 - DNA, 1467 bp, synthetic construct
  misc_feature 1..1467: note = Description of Artificial Sequence: Syntheticpolynucleotide
  source 1..1467: mol_type = other DNA
atggcactccccgtaactgctctgctgctgccgttggcattgctcctgcacgccgcacgcccgcaggtgcagctgcaggaatccggaccggggctggtgaagcccagcgagactctgagtctcacgtgtacagtttctggaggtagcattagctcctactattggtcatggataaggcagccccccgggaagggattggaatggatcggctatatttactacagtgggagcaccaattacaacccctcactgaagtctagagttacaatcagcgttgacacctcaaagaatcagttcagtttgaaattgtctagcgtcacagcagctgatacagccgtctattattgtgtttctctggtctattgcggtggggattgttacagtggctttgactattgggggcagggtactctggttacagtttcttccggggggggaggctctgggggcggaggctcaggtggtggaggcagcgacatccagttgacacagagcccgagttccttgtccgcctccgtcggggatagagtgtcatttacctgtcaggcctctcaggatattaataactttctgaattggtatcagcaaaagcccggaaaggcacccaagctgttgatttacgacgccagtaacctggagacaggcgtgccctcccggtttagtggtagcggaagcggtacggattttacctttactatcagctctctccaacccgaagacattgcaacctactattgtcaacaatatggaaacctgccttttacatttggcggcggcaccaaggtggagattaagcgggcggcagctattgaggtgatgtatccaccgccttacctggataacgaaaagagtaacggtaccatcattcacgtgaaaggtaaacacctgtgtccttctcccctcttccccgggccatcaaagcccttctgggttcttgtggtcgtgggaggcgtgcttgcttgttattctctgctcgttaccgtggcgtttatcattttttgggttagatccaaaagaagccgcctgctccatagcgattacatgaatatgactccacgccgccctggccccacaaggaaacactaccagccttacgcaccacctagagatttcgctgcctatcggagcagggtgaagttttccagatctgcagatgcaccagcgtatcagcagggccagaaccaactgtataacgagctcaacctgggacgcagggaagagtatgacgttttggacaagcgcagaggacgggaccctgagatgggtggcaaaccaagacgaaaaaacccccaggagggtctctataatgagctgcagaaggataagatggctgaagcctattctgaaataggcatgaaaggagagcggagaaggggaaaagggcacgacggtttgtaccagggactcagcactgctacgaaggatacttatgacgctctccacatgcaagccctgccacctaggtaa

SEQ ID NO: 30 - protein, 488 aa, synthetic construct
  REGION 1..488: note = Description of Artificial Sequence: Syntheticpolypeptide
MALPVTALLLPLALLLHAARPQVQLQESGPGLVKPSETLSLTCTVSGGSISSYYWSWIRQPPGKGLEWIGYIYYSGSTNYNPSLKSRVTISVDTSKNQFSLKLSSVTAADTAVYYCVSLVYCGGDCYSGFDYWGQGTLVTVSSGGGGSGGGGSGGGGSDIQLTQSPSSLSASVGDRVSFTCQASQDINNFLNWYQQKPGKAPKLLIYDASNLETGVPSRFSGSGSGTDFTFTISSLQPEDIATYYCQQYGNLPFTFGGGTKVEIKRAAAIEVMYPPPYLDNEKSNGTIIHVKGKHLCPSPLFPGPSKPFWVLVVVGGVLACYSLLVTVAFIIFWVRSKRSRLLHSDYMNMTPRRPGPTRKHYQPYAPPRDFAAYRSRVKFSRSADAPAYQQGQNQLYNELNLGRREEYDVLDKRRGRDPEMGGKPRRKNPQEGLYNELQKDKMAEAYSEIGMKGERRRGKGHDGLYQGLSTATKDTYDALHMQALPPR

SEQ ID NO: 31 - DNA, 1401 bp, synthetic construct
  misc_feature 1..1401: note = Description of Artificial Sequence: Syntheticpolynucleotide
  source 1..1401: mol_type = other DNA
caggtgcagctgcaggaatccggaccggggctggtgaagcccagcgagactctgagtctcacgtgtacagtttctggaggtagcattagctcctactattggtcatggataaggcagccccccgggaagggattggaatggatcggctatatttactacagtgggagcaccaattacaacccctcactgaagtctagagttacaatcagcgttgacacctcaaagaatcagttcagtttgaaattgtctagcgtcacagcagctgatacagccgtctattattgtgtttctctggtctattgcggtggggattgttacagtggctttgactattgggggcagggtactctggttacagtttcttccggggggggaggctctgggggcggaggctcaggtggtggaggcagcgacatccagttgacacagagcccgagttccttgtccgcctccgtcggggatagagtgtcatttacctgtcaggcctctcaggatattaataactttctgaattggtatcagcaaaagcccggaaaggcacccaagctgttgatttacgacgccagtaacctggagacaggcgtgccctcccggtttagtggtagcggaagcggtacggattttacctttactatcagctctctccaacccgaagacattgcaacctactattgtcaacaatatggaaacctgccttttacatttggcggcggcaccaaggtggagattaagcgggcggcagctattgaggtgatgtatccaccgccttacctggataacgaaaagagtaacggtaccatcattcacgtgaaaggtaaacacctgtgtccttctcccctcttccccgggccatcaaagcccttctgggttcttgtggtcgtgggaggcgtgcttgcttgttattctctgctcgttaccgtggcgtttatcattttttgggttagatccaaaagaagccgcctgctccatagcgattacatgaatatgactccacgccgccctggccccacaaggaaacactaccagccttacgcaccacctagagatttcgctgcctatcggagcagggtgaagttttccagatctgcagatgcaccagcgtatcagcagggccagaaccaactgtataacgagctcaacctgggacgcagggaagagtatgacgttttggacaagcgcagaggacgggaccctgagatgggtggcaaaccaagacgaaaaaacccccaggagggtctctataatgagctgcagaaggataagatggctgaagcctattctgaaataggcatgaaaggagagcggagaaggggaaaagggcacgacggtttgtaccagggactcagcactgctacgaaggatacttatgacgctctccacatgcaagccctgccacctagg

SEQ ID NO: 32 - protein, 467 aa, synthetic construct
  REGION 1..467: note = Description of Artificial Sequence: Syntheticpolypeptide
QVQLQESGPGLVKPSETLSLTCTVSGGSISSYYWSWIRQPPGKGLEWIGYIYYSGSTNYNPSLKSRVTISVDTSKNQFSLKLSSVTAADTAVYYCVSLVYCGGDCYSGFDYWGQGTLVTVSSGGGGSGGGGSGGGGSDIQLTQSPSSLSASVGDRVSFTCQASQDINNFLNWYQQKPGKAPKLLIYDASNLETGVPSRFSGSGSGTDFTFTISSLQPEDIATYYCQQYGNLPFTFGGGTKVEIKRAAAIEVMYPPPYLDNEKSNGTIIHVKGKHLCPSPLFPGPSKPFWVLVVVGGVLACYSLLVTVAFIIFWVRSKRSRLLHSDYMNMTPRRPGPTRKHYQPYAPPRDFAAYRSRVKFSRSADAPAYQQGQNQLYNELNLGRREEYDVLDKRRGRDPEMGGKPRRKNPQEGLYNELQKDKMAEAYSEIGMKGERRRGKGHDGLYQGLSTATKDTYDALHMQALPPR

SEQ ID NO: 33 - DNA, 1548 bp, synthetic construct
  misc_feature 1..1548: note = Description of Artificial Sequence: Syntheticpolynucleotide
  source 1..1548: mol_type = other DNA
atggcactccccgtaactgctctgctgctgccgttggcattgctcctgcacgccgcacgcccgcaggtgcaattgcaagagtccggccccggactcgttaaacccagtgagacgcttagcctgacctgtaccgtctcagggggcagcatctcctcttattactggagctggatcaggcagcctccaggaaaaggccttgaatggattgggtacatctactactctggctcaacaaattataatccatccctgaagtcccgcgtgactatctctgtggacaccagcaagaatcagttttcactgaagttgtctagtgttaccgcggccgacaccgccgtatactactgtgtgtctcttgtgtactgtggcggcgactgctattccgggttcgactactggggccaagggactctggtaaccgtgtcctcaggcggcggcgggtcaggaggaggcggcagtggaggtggcggctccgacatccagctgacacaatcaccatcttccctttcagcttcagtcggggacagagtgtccttcacatgccaggccagccaggatatcaataacttcctgaactggtaccaacagaaacccggaaaggctccaaagctcctgatctatgatgcttccaacctggagaccggcgtgccctccaggttcagtggttcaggatcaggcactgactttacgttcaccatatccagtcttcagcccgaagacattgcaacctattactgccaacaatacgggaaccttccctttacattcggaggcggcaccaaggtggaaatcaaaagggctgcagcattgagcaactcaataatgtattttagtcactttgtaccagtgttcttgccggctaagcctactaccacacccgctccacggccacctaccccagctcctaccatcgcttcacagcctctgtccctgcgcccagaggcttgccgaccggccgcagggggcgctgttcataccagaggactggatttcgcctgcgatatctatatctgggcacccctggccggaacctgcggcgtactcctgctgtccctggtcatcacgctctattgtaatcacaggaacagatccaaaagaagccgcctgctccatagcgattacatgaatatgactccacgccgccctggccccacaaggaaacactaccagccttacgcaccacctagagatttcgctgcctatcggagcagggtgaagttttccagatctgcagatgcaccagcgtatcagcagggccagaaccaactgtataacgagctcaacctgggacgcagggaagagtatgacgttttggacaagcgcagaggacgggaccctgagatgggtggcaaaccaagacgaaaaaacccccaggagggtctctataatgagctgcagaaggataagatggctgaagcctattctgaaataggcatgaaaggagagcggagaaggggaaaagggcacgacggtttgtaccagggactcagcactgctacgaaggatacttatgacgctctccacatgcaagccctgccacctaggtaa

SEQ ID NO: 34 - protein, 515 aa, synthetic construct
  REGION 1..515: note = Description of Artificial Sequence: Syntheticpolypeptide
MALPVTALLLPLALLLHAARPQVQLQESGPGLVKPSETLSLTCTVSGGSISSYYWSWIRQPPGKGLEWIGYIYYSGSTNYNPSLKSRVTISVDTSKNQFSLKLSSVTAADTAVYYCVSLVYCGGDCYSGFDYWGQGTLVTVSSGGGGSGGGGSGGGGSDIQLTQSPSSLSASVGDRVSFTCQASQDINNFLNWYQQKPGKAPKLLIYDASNLETGVPSRFSGSGSGTDFTFTISSLQPEDIATYYCQQYGNLPFTFGGGTKVEIKRAAALSNSIMYFSHFVPVFLPAKPTTTPAPRPPTPAPTIASQPLSLRPEACRPAAGGAVHTRGLDFACDIYIWAPLAGTCGVLLLSLVITLYCNHRNRSKRSRLLHSDYMNMTPRRPGPTRKHYQPYAPPRDFAAYRSRVKFSRSADAPAYQQGQNQLYNELNLGRREEYDVLDKRRGRDPEMGGKPRRKNPQEGLYNELQKDKMAEAYSEIGMKGERRRGKGHDGLYQGLSTATKDTYDALHMQALPPR

SEQ ID NO: 35 - DNA, 1482 bp, synthetic construct
  misc_feature 1..1482: note = Description of Artificial Sequence: Syntheticpolynucleotide
  source 1..1482: mol_type = other DNA
caggtgcaattgcaagagtccggccccggactcgttaaacccagtgagacgcttagcctgacctgtaccgtctcagggggcagcatctcctcttattactggagctggatcaggcagcctccaggaaaaggccttgaatggattgggtacatctactactctggctcaacaaattataatccatccctgaagtcccgcgtgactatctctgtggacaccagcaagaatcagttttcactgaagttgtctagtgttaccgcggccgacaccgccgtatactactgtgtgtctcttgtgtactgtggcggcgactgctattccgggttcgactactggggccaagggactctggtaaccgtgtcctcaggcggcggcgggtcaggaggaggcggcagtggaggtggcggctccgacatccagctgacacaatcaccatcttccctttcagcttcagtcggggacagagtgtccttcacatgccaggccagccaggatatcaataacttcctgaactggtaccaacagaaacccggaaaggctccaaagctcctgatctatgatgcttccaacctggagaccggcgtgccctccaggttcagtggttcaggatcaggcactgactttacgttcaccatatccagtcttcagcccgaagacattgcaacctattactgccaacaatacgggaaccttccctttacattcggaggcggcaccaaggtggaaatcaaaagggctgcagcattgagcaactcaataatgtattttagtcactttgtaccagtgttcttgccggctaagcctactaccacacccgctccacggccacctaccccagctcctaccatcgcttcacagcctctgtccctgcgcccagaggcttgccgaccggccgcagggggcgctgttcataccagaggactggatttcgcctgcgatatctatatctgggcacccctggccggaacctgcggcgtactcctgctgtccctggtcatcacgctctattgtaatcacaggaacagatccaaaagaagccgcctgctccatagcgattacatgaatatgactccacgccgccctggccccacaaggaaacactaccagccttacgcaccacctagagatttcgctgcctatcggagcagggtgaagttttccagatctgcagatgcaccagcgtatcagcagggccagaaccaactgtataacgagctcaacctgggacgcagggaagagtatgacgttttggacaagcgcagaggacgggaccctgagatgggtggcaaaccaagacgaaaaaacccccaggagggtctctataatgagctgcagaaggataagatggctgaagcctattctgaaataggcatgaaaggagagcggagaaggggaaaagggcacgacggtttgtaccagggactcagcactgctacgaaggatacttatgacgctctccacatgcaagccctgccacctagg

SEQ ID NO: 36 - protein, 494 aa, synthetic construct
  REGION 1..494: note = Description of Artificial Sequence: Syntheticpolypeptide
QVQLQESGPGLVKPSETLSLTCTVSGGSISSYYWSWIRQPPGKGLEWIGYIYYSGSTNYNPSLKSRVTISVDTSKNQFSLKLSSVTAADTAVYYCVSLVYCGGDCYSGFDYWGQGTLVTVSSGGGGSGGGGSGGGGSDIQLTQSPSSLSASVGDRVSFTCQASQDINNFLNWYQQKPGKAPKLLIYDASNLETGVPSRFSGSGSGTDFTFTISSLQPEDIATYYCQQYGNLPFTFGGGTKVEIKRAAALSNSIMYFSHFVPVFLPAKPTTTPAPRPPTPAPTIASQPLSLRPEACRPAAGGAVHTRGLDFACDIYIWAPLAGTCGVLLLSLVITLYCNHRNRSKRSRLLHSDYMNMTPRRPGPTRKHYQPYAPPRDFAAYRSRVKFSRSADAPAYQQGQNQLYNELNLGRREEYDVLDKRRGRDPEMGGKPRRKNPQEGLYNELQKDKMAEAYSEIGMKGERRRGKGHDGLYQGLSTATKDTYDALHMQALPPR

SEQ ID NO: 37 - DNA, 1440 bp, synthetic construct
  misc_feature 1..1440: note = Description of Artificial Sequence: Syntheticpolynucleotide
  source 1..1440: mol_type = other DNA
atggcactccccgtaactgctctgctgctgccgttggcattgctcctgcacgccgcacgcccggatatccagctcacgcaatccccctcaagcttgagtgcctccgtgggcgaccgggtgtccttcacatgtcaggcaagccaagacataaataatttcctgaattggtaccaacaaaaacccggcaaggctcccaaactcctgatttatgatgcctccaatctggagaccggggtcccttctagattcagcggaagtggcagcggcacagactttacatttactatctcttctctgcaaccagaggacatcgccacatactattgccagcaatacggcaatctgcccttcaccttcggaggcggaaccaaggtagaaattaaaaggggcggtggaggctccggaggggggggctctggcggagggggctcccaagtacaattgcaggagtcagggcctggactcgtgaagccttcagaaactttgtcactgacatgtacagtgtccggcggaagcatttccagttactattggtcctggattagacagccacccggcaaaggactggaatggattggatatatctactactctggatctacaaactataatcccagcctcaaatccagggtcactattagtgtggatacatcaaagaatcagttctccttgaagctgagctcagtcactgctgccgacaccgcagtgtactattgtgtgagcctggtctactgcggcggagattgctacagcggtttcgattactggggccagggcaccctggttaccgttagttccgcggctgctcttgataacgagaagtccaacggtacgattatccacgttaagggtaagcacctttgccctagcccgctgttcccaggccccagtaagcccttttgggtcctcgttgtggtaggtggggtactcgcctgctactccctgctcgtcactgtcgcattcatcatcttctgggtcagatccaaaagaagccgcctgctccatagcgattacatgaatatgactccacgccgccctggccccacaaggaaacactaccagccttacgcaccacctagagatttcgctgcctatcggagcagggtgaagttttccagatctgcagatgcaccagcgtatcagcagggccagaaccaactgtataacgagctcaacctgggacgcagggaagagtatgacgttttggacaagcgcagaggacgggaccctgagatgggtggcaaaccaagacgaaaaaacccccaggagggtctctataatgagctgcagaaggataagatggctgaagcctattctgaaataggcatgaaaggagagcggagaaggggaaaagggcacgacggtttgtaccagggactcagcactgctacgaaggatacttatgacgctctccacatgcaagccctgccacctaggtaa

SEQ ID NO: 38 - protein, 458 aa, synthetic construct
  REGION 1..458: note = Description of Artificial Sequence: Syntheticpolypeptide
DIQLTQSPSSLSASVGDRVSFTCQASQDINNFLNWYQQKPGKAPKLLIYDASNLETGVPSRFSGSGSGTDFTFTISSLQPEDIATYYCQQYGNLPFTFGGGTKVEIKRGGGGSGGGGSGGGGSQVQLQESGPGLVKPSETLSLTCTVSGGSISSYYWSWIRQPPGKGLEWIGYIYYSGSTNYNPSLKSRVTISVDTSKNQFSLKLSSVTAADTAVYYCVSLVYCGGDCYSGFDYWGQGTLVTVSSAAALDNEKSNGTIIHVKGKHLCPSPLFPGPSKPFWVLVVVGGVLACYSLLVTVAFIIFWVRSKRSRLLHSDYMNMTPRRPGPTRKHYQPYAPPRDFAAYRSRVKFSRSADAPAYQQGQNQLYNELNLGRREEYDVLDKRRGRDPEMGGKPRRKNPQEGLYNELQKDKMAEAYSEIGMKGERRRGKGHDGLYQGLSTATKDTYDALHMQALPPR

SEQ ID NO: 39 - DNA, 1374 bp, synthetic construct
  misc_feature 1..1374: note = Description of Artificial Sequence: Syntheticpolynucleotide
  source 1..1374: mol_type = other DNA
gatatccagctcacgcaatccccctcaagcttgagtgcctccgtgggcgaccgggtgtccttcacatgtcaggcaagccaagacataaataatttcctgaattggtaccaacaaaaacccggcaaggctcccaaactcctgatttatgatgcctccaatctggagaccggggtcccttctagattcagcggaagtggcagcggcacagactttacatttactatctcttctctgcaaccagaggacatcgccacatactattgccagcaatacggcaatctgcccttcaccttcggaggcggaaccaaggtagaaattaaaaggggcggtggaggctccggaggggggggctctggcggagggggctcccaagtacaattgcaggagtcagggcctggactcgtgaagccttcagaaactttgtcactgacatgtacagtgtccggcggaagcatttccagttactattggtcctggattagacagccacccggcaaaggactggaatggattggatatatctactactctggatctacaaactataatcccagcctcaaatccagggtcactattagtgtggatacatcaaagaatcagttctccttgaagctgagctcagtcactgctgccgacaccgcagtgtactattgtgtgagcctggtctactgcggcggagattgctacagcggtttcgattactggggccagggcaccctggttaccgttagttccgcggctgctcttgataacgagaagtccaacggtacgattatccacgttaagggtaagcacctttgccctagcccgctgttcccaggccccagtaagcccttttgggtcctcgttgtggtaggtggggtactcgcctgctactccctgctcgtcactgtcgcattcatcatcttctgggtcagatccaaaagaagccgcctgctccatagcgattacatgaatatgactccacgccgccctggccccacaaggaaacactaccagccttacgcaccacctagagatttcgctgcctatcggagcagggtgaagttttccagatctgcagatgcaccagcgtatcagcagggccagaaccaactgtataacgagctcaacctgggacgcagggaagagtatgacgttttggacaagcgcagaggacgggaccctgagatgggtggcaaaccaagacgaaaaaacccccaggagggtctctataatgagctgcagaaggataagatggctgaagcctattctgaaataggcatgaaaggagagcggagaaggggaaaagggcacgacggtttgtaccagggactcagcactgctacgaaggatacttatgacgctctccacatgcaagccctgccacctagg

SEQ ID NO: 40 - protein, 458 aa, synthetic construct; identical to SEQ ID NO: 38
  REGION 1..458: note = Description of Artificial Sequence: Syntheticpolypeptide

SEQ ID NO: 41 - DNA, 1467 bp, synthetic construct
  misc_feature 1..1467: note = Description of Artificial Sequence: Syntheticpolynucleotide
  source 1..1467: mol_type = other DNA
atggcactccccgtaactgctctgctgctgccgttggcattgctcctgcacgccgcacgcccggatatccagctgacccagtctccatcctctttgagtgcctccgtgggtgaccgcgtctctttcacttgccaagccagccaagacatcaacaactttctgaattggtaccagcagaaaccaggcaaagcaccaaagctcctcatctacgacgcctccaacctggaaaccggggtgcccagcaggtttagcgggagcggttctggcacggattttacgttcaccatctcctctctgcagcccgaggatatagctacttattactgtcagcagtacgggaatctgccatttacttttgggggtggaactaaggtggaaatcaaaaggggcggcgggggaagcgggggcgggggctcaggtggcggagggagccaggtgcaactccaggaaagtggcccaggattggtgaagcccagcgagaccctttcccttacttgtactgttagcggaggcagcataagcagctactattggtcctggatcagacagccaccagggaaagggcttgaatggattggctacatttactattccgggtccaccaactacaacccatccctcaagtcccgcgtgacaatttccgtcgacacaagcaagaaccagttctccctgaaacttagtagcgtcactgctgcagatacagcagtgtactattgtgtcagccttgtctactgtggcggcgactgctacagtggctttgattactggggacagggcacgctcgtgacagtgtccagcgctgcggctatcgaggtaatgtatccgccaccgtatctggacaacgagaagtctaatgggacaatcattcacgtgaaggggaagcacctgtgtccatcccccctgtttccgggtcccagtaaacccttctgggtgcttgttgtcgttggcggggtgctggcctgctattccctgctggtgaccgtcgcgtttattattttctgggttagatccaaaagaagccgcctgctccatagcgattacatgaatatgactccacgccgccctggccccacaaggaaacactaccagccttacgcaccacctagagatttcgctgcctatcggagcagggtgaagttttccagatctgcagatgcaccagcgtatcagcagggccagaaccaactgtataacgagctcaacctgggacgcagggaagagtatgacgttttggacaagcgcagaggacgggaccctgagatgggtggcaaaccaagacgaaaaaacccccaggagggtctctataatgagctgcagaaggataagatggctgaagcctattctgaaataggcatgaaaggagagcggagaaggggaaaagggcacgacggtttgtaccagggactcagcactgctacgaaggatacttatgacgctctccacatgcaagccctgccacctaggtaa

SEQ ID NO: 42 - protein, 488 aa, synthetic construct
  REGION 1..488: note = Description of Artificial Sequence: Syntheticpolypeptide
MALPVTALLLPLALLLHAARPDIQLTQSPSSLSASVGDRVSFTCQASQDINNFLNWYQQKPGKAPKLLIYDASNLETGVPSRFSGSGSGTDFTFTISSLQPEDIATYYCQQYGNLPFTFGGGTKVEIKRGGGGSGGGGSGGGGSQVQLQESGPGLVKPSETLSLTCTVSGGSISSYYWSWIRQPPGKGLEWIGYIYYSGSTNYNPSLKSRVTISVDTSKNQFSLKLSSVTAADTAVYYCVSLVYCGGDCYSGFDYWGQGTLVTVSSAAAIEVMYPPPYLDNEKSNGTIIHVKGKHLCPSPLFPGPSKPFWVLVVVGGVLACYSLLVTVAFIIFWVRSKRSRLLHSDYMNMTPRRPGPTRKHYQPYAPPRDFAAYRSRVKFSRSADAPAYQQGQNQLYNELNLGRREEYDVLDKRRGRDPEMGGKPRRKNPQEGLYNELQKDKMAEAYSEIGMKGERRRGKGHDGLYQGLSTATKDTYDALHMQALPPR

SEQ ID NO: 43 - DNA, 1401 bp, synthetic construct
  misc_feature 1..1401: note = Description of Artificial Sequence: Syntheticpolynucleotide
  source 1..1401: mol_type = other DNA
gatatccagctgacccagtctccatcctctttgagtgcctccgtgggtgaccgcgtctctttcacttgccaagccagccaagacatcaacaactttctgaattggtaccagcagaaaccaggcaaagcaccaaagctcctcatctacgacgcctccaacctggaaaccggggtgcccagcaggtttagcgggagcggttctggcacggattttacgttcaccatctcctctctgcagcccgaggatatagctacttattactgtcagcagtacgggaatctgccatttacttttgggggtggaactaaggtggaaatcaaaaggggcggcgggggaagcgggggcgggggctcaggtggcggagggagccaggtgcaactccaggaaagtggcccaggattggtgaagcccagcgagaccctttcccttacttgtactgttagcggaggcagcataagcagctactattggtcctggatcagacagccaccagggaaagggcttgaatggattggctacatttactattccgggtccaccaactacaacccatccctcaagtcccgcgtgacaatttccgtcgacacaagcaagaaccagttctccctgaaacttagtagcgtcactgctgcagatacagcagtgtactattgtgtcagccttgtctactgtggcggcgactgctacagtggctttgattactggggacagggcacgctcgtgacagtgtccagcgctgcggctatcgaggtaatgtatccgccaccgtatctggacaacgagaagtctaatgggacaatcattcacgtgaaggggaagcacctgtgtccatcccccctgtttccgggtcccagtaaacccttctgggtgcttgttgtcgttggcggggtgctggcctgctattccctgctggtgaccgtcgcgtttattattttctgggttagatccaaaagaagccgcctgctccatagcgattacatgaatatgactccacgccgccctggccccacaaggaaacactaccagccttacgcaccacctagagatttcgctgcctatcggagcagggtgaagttttccagatctgcagatgcaccagcgtatcagcagggccagaaccaactgtataacgagctcaacctgggacgcagggaagagtatgacgttttggacaagcgcagaggacgggaccctgagatgggtggcaaaccaagacgaaaaaacccccaggagggtctctataatgagctgcagaaggataagatggctgaagcctattctgaaataggcatgaaaggagagcggagaaggggaaaagggcacgacggtttgtaccagggactcagcactgctacgaaggatacttatgacgctctccacatgcaagccctgccacctagg

SEQ ID NO: 44 - protein, 467 aa, synthetic construct
  REGION 1..467: note = Description of Artificial Sequence: Syntheticpolypeptide
DIQLTQSPSSLSASVGDRVSFTCQASQDINNFLNWYQQKPGKAPKLLIYDASNLETGVPSRFSGSGSGTDFTFTISSLQPEDIATYYCQQYGNLPFTFGGGTKVEIKRGGGGSGGGGSGGGGSQVQLQESGPGLVKPSETLSLTCTVSGGSISSYYWSWIRQPPGKGLEWIGYIYYSGSTNYNPSLKSRVTISVDTSKNQFSLKLSSVTAADTAVYYCVSLVYCGGDCYSGFDYWGQGTLVTVSSAAAIEVMYPPPYLDNEKSNGTIIHVKGKHLCPSPLFPGPSKPFWVLVVVGGVLACYSLLVTVAFIIFWVRSKRSRLLHSDYMNMTPRRPGPTRKHYQPYAPPRDFAAYRSRVKFSRSADAPAYQQGQNQLYNELNLGRREEYDVLDKRRGRDPEMGGKPRRKNPQEGLYNELQKDKMAEAYSEIGMKGERRRGKGHDGLYQGLSTATKDTYDALHMQALPPR

SEQ ID NO: 45 - DNA, 1548 bp, synthetic construct
  misc_feature 1..1548: note = Description of Artificial Sequence: Syntheticpolynucleotide
  source 1..1548: mol_type = other DNA
atggcactccccgtaactgctctgctgctgccgttggcattgctcctgcacgccgcacgcccggacattcaattgacccagtcccctagcagtctctcagcaagtgtgggagatagggtgtcattcacctgtcaggcttcacaggacatcaacaacttcctcaattggtatcagcagaagccagggaaggcaccaaagctgctcatatatgacgcttcaaaccttgaaaccggagtacctagccgcttcagcggaagcggatcagggactgacttcacttttaccatctcttcactgcagcccgaagacatcgccacatactactgccagcagtacggaaacttgccttttacatttgggggcggcaccaaagtggagattaagcgagggggaggcggctcaggaggcggtggctccggaggcgggggttcccaggtccagctccaggaatccggcccaggtctggttaagcccagtgaaactttgtccctcacgtgtactgtgagcggtggttcaatctcctcatactattggtcttggatacggcaacctcctggaaagggcctcgagtggatcggctatatctactatagtggctccactaattacaacccttccctcaagtccagagtcaccatttccgtggacacatctaagaaccagttcagtctgaagttgtccagcgttacagccgcagacacagccgtttattactgtgtgtctcttgtttactgcgggggagactgttatagcggcttcgattactggggccagggcaccttggtcacagtctcttccgcggccgccctctctaacagtattatgtacttttctcattttgtacccgtgttccttcccgctaagccaactactaccccggccccacggccgcctacccctgcacccacaatagccagtcagcctttgagcctgagacctgaggcttgtcggccggctgctgggggtgcagtgcacacacgaggtcttgattttgcttgcgacatatacatctgggcccctctggccgggacctgtggggtgctgcttctgagcttggtcatcacgctctattgcaaccatcgcaacagatccaaaagaagccgcctgctccatagcgattacatgaatatgactccacgccgccctggccccacaaggaaacactaccagccttacgcaccacctagagatttcgctgcctatcggagcagggtgaagttttccagatctgcagatgcaccagcgtatcagcagggccagaaccaactgtataacgagctcaacctgggacgcagggaagagtatgacgttttggacaagcgcagaggacgggaccctgagatgggtggcaaaccaagacgaaaaaacccccaggagggtctctataatgagctgcagaaggataagatggctgaagcctattctgaaataggcatgaaaggagagcggagaaggggaaaagggcacgacggtttgtaccagggactcagcactgctacgaaggatacttatgacgctctccacatgcaagccctgccacctaggtaa

SEQ ID NO: 46 - protein, 515 aa, synthetic construct
  REGION 1..515: note = Description of Artificial Sequence: Syntheticpolypeptide
MALPVTALLLPLALLLHAARPDIQLTQSPSSLSASVGDRVSFTCQASQDINNFLNWYQQKPGKAPKLLIYDASNLETGVPSRFSGSGSGTDFTFTISSLQPEDIATYYCQQYGNLPFTFGGGTKVEIKRGGGGSGGGGSGGGGSQVQLQESGPGLVKPSETLSLTCTVSGGSISSYYWSWIRQPPGKGLEWIGYIYYSGSTNYNPSLKSRVTISVDTSKNQFSLKLSSVTAADTAVYYCVSLVYCGGDCYSGFDYWGQGTLVTVSSAAALSNSIMYFSHFVPVFLPAKPTTTPAPRPPTPAPTIASQPLSLRPEACRPAAGGAVHTRGLDFACDIYIWAPLAGTCGVLLLSLVITLYCNHRNRSKRSRLLHSDYMNMTPRRPGPTRKHYQPYAPPRDFAAYRSRVKFSRSADAPAYQQGQNQLYNELNLGRREEYDVLDKRRGRDPEMGGKPRRKNPQEGLYNELQKDKMAEAYSEIGMKGERRRGKGHDGLYQGLSTATKDTYDALHMQALPPR

SEQ ID NO: 47 - DNA, 1482 bp, synthetic construct
  misc_feature 1..1482: note = Description of Artificial Sequence: Syntheticpolynucleotide
  source 1..1482: mol_type = other DNA
gacattcaattgacccagtcccctagcagtctctcagcaagtgtgggagatagggtgtcattcacctgtcaggcttcacaggacatcaacaacttcctcaattggtatcagcagaagccagggaaggcaccaaagctgctcatatatgacgcttcaaaccttgaaaccggagtacctagccgcttcagcggaagcggatcagggactgacttcacttttaccatctcttcactgcagcccgaagacatcgccacatactactgccagcagtacggaaacttgccttttacatttgggggcggcaccaaagtggagattaagcgagggggaggcggctcaggaggcggtggctccggaggcgggggttcccaggtccagctccaggaatccggcccaggtctggttaagcccagtgaaactttgtccctcacgtgtactgtgagcggtggttcaatctcctcatactattggtcttggatacggcaacctcctggaaagggcctcgagtggatcggctatatctactatagtggctccactaattacaacccttccctcaagtccagagtcaccatttccgtggacacatctaagaaccagttcagtctgaagttgtccagcgttacagccgcagacacagccgtttattactgtgtgtctcttgtttactgcgggggagactgttatagcggcttcgattactggggccagggcaccttggtcacagtctcttccgcggccgccctctctaacagtattatgtacttttctcattttgtacccgtgttccttcccgctaagccaactactaccccggccccacggccgcctacccctgcacccacaatagccagtcagcctttgagcctgagacctgaggcttgtcggccggctgctgggggtgcagtgcacacacgaggtcttgattttgcttgcgacatatacatctgggcccctctggccgggacctgtggggtgctgcttctgagcttggtcatcacgctctattgcaaccatcgcaacagatccaaaagaagccgcctgctccatagcgattacatgaatatgactccacgccgccctggccccacaaggaaacactaccagccttacgcaccacctagagatttcgctgcctatcggagcagggtgaagttttccagatctgcagatgcaccagcgtatcagcagggccagaaccaactgtataacgagctcaacctgggacgcagggaagagtatgacgttttggacaagcgcagaggacgggaccctgagatgggtggcaaaccaagacgaaaaaacccccaggagggtctctataatgagctgcagaaggataagatggctgaagcctattctgaaataggcatgaaaggagagcggagaaggggaaaagggcacgacggtttgtaccagggactcagcactgctacgaaggatacttatgacgctctccacatgcaagccctgccacctagg

SEQ ID NO: 48 - protein, 494 aa, synthetic construct
  REGION 1..494: note = Description of Artificial Sequence: Syntheticpolypeptide
DIQLTQSPSSLSASVGDRVSFTCQASQDINNFLNWYQQKPGKAPKLLIYDASNLETGVPSRFSGSGSGTDFTFTISSLQPEDIATYYCQQYGNLPFTFGGGTKVEIKRGGGGSGGGGSGGGGSQVQLQESGPGLVKPSETLSLTCTVSGGSISSYYWSWIRQPPGKGLEWIGYIYYSGSTNYNPSLKSRVTISVDTSKNQFSLKLSSVTAADTAVYYCVSLVYCGGDCYSGFDYWGQGTLVTVSSAAALSNSIMYFSHFVPVFLPAKPTTTPAPRPPTPAPTIASQPLSLRPEACRPAAGGAVHTRGLDFACDIYIWAPLAGTCGVLLLSLVITLYCNHRNRSKRSRLLHSDYMNMTPRRPGPTRKHYQPYAPPRDFAAYRSRVKFSRSADAPAYQQGQNQLYNELNLGRREEYDVLDKRRGRDPEMGGKPRRKNPQEGLYNELQKDKMAEAYSEIGMKGERRRGKGHDGLYQGLSTATKDTYDALHMQALPPR

SEQ ID NO: 49 - DNA, 372 bp, synthetic construct
  misc_feature 1..372: note = Description of Artificial Sequence: Syntheticpolynucleotide
  source 1..372: mol_type = other DNA
caggtacagctgcaggaatctgggcccggacttgtcaagccaagtcagacactttctcttacatgtaccgtgagcggcggaagtataagcagtggaggcttttactggtcttggatacggcagcacccaggcaaaggcttggagtggattggatacattcatcattcaggatctacacactataatccatcccttaagtcccgggtcaccattagcattgatacgtctaagaatctgttcagtctcaggctgtcctccgtcactgctgccgacacagccgtgtactactgcgcctccttggtttactgcggaggcgactgttatagcggctttgattattgggggcaggggaccctcgtaaccgtgagctct

SEQ ID NO: 50 - protein, 124 aa, synthetic construct
  REGION 1..124: note = Description of Artificial Sequence: Syntheticpolypeptide
QVQLQESGPGLVKPSQTLSLTCTVSGGSISSGGFYWSWIRQHPGKGLEWIGYIHHSGSTHYNPSLKSRVTISIDTSKNLFSLRLSSVTAADTAVYYCASLVYCGGDCYSGFDYWGQGTLVTVSS

SEQ ID NO: 51 - protein, 9 aa, synthetic construct
  REGION 1..9: note = Description of Artificial Sequence: Syntheticpeptide
GGSISSGGF

SEQ ID NO: 52 - protein, 5 aa, synthetic construct
  REGION 1..5: note = Description of Artificial Sequence: Syntheticpeptide
HHSGS

SEQ ID NO: 53 - protein, 14 aa, synthetic construct
  REGION 1..14: note = Description of Artificial Sequence: Syntheticpeptide
LVYCGGDCYSGFDY

SEQ ID NO: 54 - DNA, 324 bp, synthetic construct
  misc_feature 1..324: note = Description of Artificial Sequence: Syntheticpolynucleotide
  source 1..324: mol_type = other DNA
gatatccagctcactcaaagcccctctagtctctctgcctcagtgggggatcgggtcagttttacttgtcaagcttcacaggatatcaacaacttccttaattggtatcagcagaagccaggaaaagcacccaagctgctcatctatgatgcctcaaatttggagacgggtgttcccagtcgattctctgggtcagggtccgggaccgactttacgtttacgatctcctctctgcagcccgaagacatcgccacatactattgtcaacagtacggcaacttgcctttcacatttgggggcgggactaaggttgaaatcaagagg

SEQ ID NO: 55 - protein, 108 aa, synthetic construct; identical to SEQ ID NO: 21
  REGION 1..108: note = Description of Artificial Sequence: Syntheticpolypeptide

SEQ ID NO: 56 - protein, 11 aa, synthetic construct
  REGION 1..11: note = Description of Artificial Sequence: Syntheticpeptide
QASQDINNFLN

SEQ ID NO: 57 - protein, 7 aa, synthetic construct
  REGION 1..7: note = Description of Artificial Sequence: Syntheticpeptide
DASNLET

SEQ ID NO: 58 - protein, 9 aa, synthetic construct
  REGION 1..9: note = Description of Artificial Sequence: Syntheticpeptide
QQYGNLPFT

SEQ ID NO: 59 - DNA, 1446 bp, synthetic construct
  misc_feature 1..1446: note = Description of Artificial Sequence: Syntheticpolynucleotide
  source 1..1446: mol_type = other DNA
atggcactccccgtaactgctctgctgctgccgttggcattgctcctgcacgccgcacgcccgcaggtacagctgcaggaatctgggcccggacttgtcaagccaagtcagacactttctcttacatgtaccgtgagcggcggaagtataagcagtggaggcttttactggtcttggatacggcagcacccaggcaaaggcttggagtggattggatacattcatcattcaggatctacacactataatccatcccttaagtcccgggtcaccattagcattgatacgtctaagaatctgttcagtctcaggctgtcctccgtcactgctgccgacacagccgtgtactactgcgcctccttggtttactgcggaggcgactgttatagcggctttgattattgggggcaggggaccctcgtaaccgtgagctctggagggggtgggagcgggggaggaggttcaggggggggcggctccgatatccagctcactcaaagcccctctagtctctctgcctcagtgggggatcgggtcagttttacttgtcaagcttcacaggatatcaacaacttccttaattggtatcagcagaagccaggaaaagcacccaagctgctcatctatgatgcctcaaatttggagacgggtgttcccagtcgattctctgggtcagggtccgggaccgactttacgtttacgatctcctctctgcagcccgaagacatcgccacatactattgtcaacagtacggcaacttgcctttcacatttgggggcgggactaaggttgaaatcaagagggccgctgcactggacaatgagaagtccaacggcaccatcatccacgtgaagggcaagcacctgtgccctagtcctctgttcccaggcccatccaaacctttttgggttcttgttgtggtcgggggggtgctggcctgctattctctgctggtcacggtggccttcataattttctgggttagatccaaaagaagccgcctgctccatagcgattacatgaatatgactccacgccgccctggccccacaaggaaacactaccagccttacgcaccacctagagatttcgctgcctatcggagcagggtgaagttttccagatctgcagatgcaccagcgtatcagcagggccagaaccaactgtataacgagctcaacctgggacgcagggaagagtatgacgttttggacaagcgcagaggacgggaccctgagatgggtggcaaaccaagacgaaaaaacccccaggagggtctctataatgagctgcagaaggataagatggctgaagcctattctgaaataggcatgaaaggagagcggagaaggggaaaagggcacgacggtttgtaccagggactcagcactgctacgaaggatacttatgacgctctccacatgcaagccctgccacctaggtaa

SEQ ID NO: 60 - protein, 481 aa, synthetic construct
  REGION 1..481: note = Description of Artificial Sequence: Syntheticpolypeptide
MALPVTALLLPLALLLHAARPQVQLQESGPGLVKPSQTLSLTCTVSGGSISSGGFYWSWIRQHPGKGLEWIGYIHHSGSTHYNPSLKSRVTISIDTSKNLFSLRLSSVTAADTAVYYCASLVYCGGDCYSGFDYWGQGTLVTVSSGGGGSGGGGSGGGGSDIQLTQSPSSLSASVGDRVSFTCQASQDINNFLNWYQQKPGKAPKLLIYDASNLETGVPSRFSGSGSGTDFTFTISSLQPEDIATYYCQQYGNLPFTFGGGTKVEIKRAAALDNEKSNGTIIHVKGKHLCPSPLFPGPSKPFWVLVVVGGVLACYSLLVTVAFIIFWVRSKRSRLLHSDYMNMTPRRPGPTRKHYQPYAPPRDFAAYRSRVKFSRSADAPAYQQGQNQLYNELNLGRREEYDVLDKRRGRDPEMGGKPRRKNPQEGLYNELQKDKMAEAYSEIGMKGERRRGKGHDGLYQGLSTATKDTYDALHMQALPPR

SEQ ID NO: 61 - DNA, 1380 bp, synthetic construct
  misc_feature 1..1380: note = Description of Artificial Sequence: Syntheticpolynucleotide
  source 1..1380: mol_type = other DNA
caggtacagctgcaggaatctgggcccggacttgtcaagccaagtcagacactttctcttacatgtaccgtgagcggcggaagtataagcagtggaggcttttactggtcttggatacggcagcacccaggcaaaggcttggagtggattggatacattcatcattcaggatctacacactataatccatcccttaagtcccgggtcaccattagcattgatacgtctaagaatctgttcagtctcaggctgtcctccgtcactgctgccgacacagccgtgtactactgcgcctccttggtttactgcggaggcgactgttatagcggctttgattattgggggcaggggaccctcgtaaccgtgagctctggagggggtgggagcgggggaggaggttcaggggggggcggctccgatatccagctcactcaaagcccctctagtctctctgcctcagtgggggatcgggtcagttttacttgtcaagcttcacaggatatcaacaacttccttaattggtatcagcagaagccaggaaaagcacccaagctgctcatctatgatgcctcaaatttggagacgggtgttcccagtcgattctctgggtcagggtccgggaccgactttacgtttacgatctcctctctgcagcccgaagacatcgccacatactattgtcaacagtacggcaacttgcctttcacatttgggggcgggactaaggttgaaatcaagagggccgctgcactggacaatgagaagtccaacggcaccatcatccacgtgaagggcaagcacctgtgccctagtcctctgttcccaggcccatccaaacctttttgggttcttgttgtggtcgggggggtgctggcctgctattctctgctggtcacggtggccttcataattttctgggttagatccaaaagaagccgcctgctccatagcgattacatgaatatgactccacgccgccctggccccacaaggaaacactaccagccttacgcaccacctagagatttcgctgcctatcggagcagggtgaagttttccagatctgcagatgcaccagcgtatcagcagggccagaaccaactgtataacgagctcaacctgggacgcagggaagagtatgacgttttggacaagcgcagaggacgggaccctgagatgggtggcaaaccaagacgaaaaaacccccaggagggtctctataatgagctgcagaaggataagatggctgaagcctattctgaaataggcatgaaaggagagcggagaaggggaaaagggcacgacggtttgtaccagggactcagcactgctacgaaggatacttatgacgctctccacatgcaagccctgccacctagg

SEQ ID NO: 62 - protein, 460 aa, synthetic construct
  REGION 1..460: note = Description of Artificial Sequence: Syntheticpolypeptide
QVQLQESGPGLVKPSQTLSLTCTVSGGSISSGGFYWSWIRQHPGKGLEWIGYIHHSGSTHYNPSLKSRVTISIDTSKNLFSLRLSSVTAADTAVYYCASLVYCGGDCYSGFDYWGQGTLVTVSSGGGGSGGGGSGGGGSDIQLTQSPSSLSASVGDRVSFTCQASQDINNFLNWYQQKPGKAPKLLIYDASNLETGVPSRFSGSGSGTDFTFTISSLQPEDIATYYCQQYGNLPFTFGGGTKVEIKRAAALDNEKSNGTIIHVKGKHLCPSPLFPGPSKPFWVLVVVGGVLACYSLLVTVAFIIFWVRSKRSRLLHSDYMNMTPRRPGPTRKHYQPYAPPRDFAAYRSRVKFSRSADAPAYQQGQNQLYNELNLGRREEYDVLDKRRGRDPEMGGKPRRKNPQEGLYNELQKDKMAEAYSEIGMKGERRRGKGHDGLYQGLSTATKDTYDALHMQALPPR

SEQ ID NO: 63 - DNA, 1473 bp, synthetic construct
  misc_feature 1..1473: note = Description of Artificial Sequence: Syntheticpolynucleotide
  source 1..1473: mol_type = other DNA
atggcactccccgtaactgctctgctgctgccgttggcattgctcctgcacgccgcacgcccgcaggtgcagctgcaggaaagcggtccgggacttgtcaagccgtcccaaacgctgagtctgacgtgtactgtctctggtggctctatttcttccgggggcttttattggtcttggatcagacaacaccctggcaaagggctggagtggatagggtatattcaccactctgggtccactcactacaacccatcattgaaatccagagtgactatctcaatcgacacatccaagaaccttttcagcctgaggttgtcatcagttaccgccgctgacaccgcggtgtattattgcgcctctctcgtgtactgcggtggcgattgttatagtggctttgactactgggggcaggggacattggttaccgtttcaagtggaggcggtgggtctggcgggggcggtagcggaggtggggggagcgacatacagcttacgcagagcccctccagcctttcagcctccgtgggggatagggtgtcctttacctgccaggcttcccaggacataaacaacttcctcaattggtatcagcaaaagcccgggaaagcaccaaagctgctcatctacgatgccagcaacctggaaaccggagtgccgtctcgcttctctggaagtggcagtgggaccgatttcacttttacaatctcaagtttgcagccagaagacattgcaacatactactgtcaacagtacggcaatctcccctttacatttggggggggaactaaagtggagattaagcgcgctgcagccattgaagttatgtatccgcccccgtatctggataacgagaaatctaatggtaccataatacatgtgaaggggaagcacctctgtccatcaccgctgttccccggcccttcaaaacctttctgggtactcgttgtcgtgggtggagttctggcctgctatagtctgctggtgaccgtggcgtttatcatcttctgggtaagatccaaaagaagccgcctgctccatagcgattacatgaatatgactccacgccgccctggccccacaaggaaacactaccagccttacgcaccacctagagatttcgctgcctatcggagcagggtgaagttttccagatctgcagatgcaccagcgtatcagcagggccagaaccaactgtataacgagctcaacctgggacgcagggaagagtatgacgttttggacaagcgcagaggacgggaccctgagatgggtggcaaaccaagacgaaaaaacccccaggagggtctctataatgagctgcagaaggataagatggctgaagcctattctgaaataggcatgaaaggagagcggagaaggggaaaagggcacgacggtttgtaccagggactcagcactgctacgaaggatacttatgacgctctccacatgcaagccctgccacctaggtaa

SEQ ID NO: 64 - protein, 490 aa, synthetic construct
  REGION 1..490: note = Description of Artificial Sequence: Syntheticpolypeptide
MALPVTALLLPLALLLHAARPQVQLQESGPGLVKPSQTLSLTCTVSGGSISSGGFYWSWIRQHPGKGLEWIGYIHHSGSTHYNPSLKSRVTISIDTSKNLFSLRLSSVTAADTAVYYCASLVYCGGDCYSGFDYWGQGTLVTVSSGGGGSGGGGSGGGGSDIQLTQSPSSLSASVGDRVSFTCQASQDINNFLNWYQQKPGKAPKLLIYDASNLETGVPSRFSGSGSGTDFTFTISSLQPEDIATYYCQQYGNLPFTFGGGTKVEIKRAAAIEVMYPPPYLDNEKSNGTIIHVKGKHLCPSPLFPGPSKPFWVLVVVGGVLACYSLLVTVAFIIFWVRSKRSRLLHSDYMNMTPRRPGPTRKHYQPYAPPRDFAAYRSRVKFSRSADAPAYQQGQNQLYNELNLGRREEYDVLDKRRGRDPEMGGKPRRKNPQEGLYNELQKDKMAEAYSEIGMKGERRRGKGHDGLYQGLSTATKDTYDALHMQALPPR

SEQ ID NO: 65 - DNA, 1407 bp, synthetic construct
  misc_feature 1..1407: note = Description of Artificial Sequence: Syntheticpolynucleotide
  source 1..1407: mol_type = other DNA
caggtgcagctgcaggaaagcggtccgggacttgtcaagccgtcccaaacgctgagtctgacgtgtactgtctctggtggctctatttcttccgggggcttttattggtcttggatcagacaacaccctggcaaagggctggagtggatagggtatattcaccactctgggtccactcactacaacccatcattgaaatccagagtgactatctcaatcgacacatccaagaaccttttcagcctgaggttgtcatcagttaccgccgctgacaccgcggtgtattattgcgcctctctcgtgtactgcggtggcgattgttatagtggctttgactactgggggcaggggacattggttaccgtttcaagtggaggcggtgggtctggcgggggcggtagcggaggtggggggagcgacatacagcttacgcagagcccctccagcctttcagcctccgtgggggatagggtgtcctttacctgccaggcttcccaggacataaacaacttcctcaattggtatcagcaaaagcccgggaaagcaccaaagctgctcatctacgatgccagcaacctggaaaccggagtgccgtctcgcttctctggaagtggcagtgggaccgatttcacttttacaatctcaagtttgcagccagaagacattgcaacatactactgtcaacagtacggcaatctcccctttacatttggggggggaactaaagtggagattaagcgcgctgcagccattgaagttatgtatccgcccccgtatctggataacgagaaatctaatggtaccataatacatgtgaaggggaagcacctctgtccatcaccgctgttccccggcccttcaaaacctttctgggtactcgttgtcgtgggtggagttctggcctgctatagtctgctggtgaccgtggcgtttatcatcttctgggtaagatccaaaagaagccgcctgctccatagcgattacatgaatatgactccacgccgccctggccccacaaggaaacactaccagccttacgcaccacctagagatttcgctgcctatcggagcagggtgaagttttccagatctgcagatgcaccagcgtatcagcagggccagaaccaactgtataacgagctcaacctgggacgcagggaagagtatgacgttttggacaagcgcagaggacgggaccctgagatgggtggcaaaccaagacgaaaaaacccccaggagggtctctataatgagctgcagaaggataagatggctgaagcctattctgaaataggcatgaaaggagagcggagaaggggaaaagggcacgacggtttgtaccagggactcagcactgctacgaaggatacttatgacgctctccacatgcaagccctgccacctagg

SEQ ID NO: 66 - protein, 469 aa, synthetic construct
  REGION 1..469: note = Description of Artificial Sequence: Syntheticpolypeptide
QVQLQESGPGLVKPSQTLSLTCTVSGGSISSGGFYWSWIRQHPGKGLEWIGYIHHSGSTHYNPSLKSRVTISIDTSKNLFSLRLSSVTAADTAVYYCASLVYCGGDCYSGFDYWGQGTLVTVSSGGGGSGGGGSGGGGSDIQLTQSPSSLSASVGDRVSFTCQASQDINNFLNWYQQKPGKAPKLLIYDASNLETGVPSRFSGSGSGTDFTFTISSLQPEDIATYYCQQYGNLPFTFGGGTKVEIKRAAAIEVMYPPPYLDNEKSNGTIIHVKGKHLCPSPLFPGPSKPFWVLVVVGGVLACYSLLVTVAFIIFWVRSKRSRLLHSDYMNMTPRRPGPTRKHYQPYAPPRDFAAYRSRVKFSRSADAPAYQQGQNQLYNELNLGRREEYDVLDKRRGRDPEMGGKPRRKNPQEGLYNELQKDKMAEAYSEIGMKGERRRGKGHDGLYQGLSTATKDTYDALHMQALPPR

SEQ ID NO: 67 - DNA, 1554 bp, synthetic construct
  misc_feature 1..1554: note = Description of Artificial Sequence: Syntheticpolynucleotide
  source 1..1554: mol_type = other DNA
atggcactccccgtaactgctctgctgctgccgttggcattgctcctgcacgccgcacgcccgcaggtgcagttgcaggaaagcgggcctggccttgtgaaaccaagccagacactgagcctgacatgcactgtgtccggcgggtccatatcttccgggggtttttattggtcctggatacgccagcatcccgggaaaggacttgaatggattggatatatccaccattccggaagcacccactacaatccaagccttaaatcccgggtgacaatctccatcgacacctcaaagaatcttttttccctgcggttgtcttcagtaactgccgccgataccgctgtgtactactgtgccagcctcgtctattgcggcggagattgttattctgggttcgattattggggtcaaggcacactggtaactgtcagcagcggaggcggcggttccgggggcgggggcagtggagggggcggatctgacattcagcttacgcagtccccatcttcacttagcgccagcgttggcgatcgggtcagcttcacgtgtcaagcaagtcaggatatcaacaactttcttaactggtaccagcagaagccaggcaaggcacccaagttgctgatttacgatgcttctaacctcgagacgggagtgcctagccgcttctccgggagcggcagcggcacagactttacctttacgatttccagtctgcagccagaggatatagcaacttattactgtcagcagtatggcaacctcccttttaccttcggtggtggcacaaaggtcgagattaaaagagccgcagcgttgtccaactccataatgtatttttctcattttgtgcccgtctttctgcctgccaaacctaccaccacccccgccccacgaccacctactccagcccccaccatcgcctcccagcccctcagcctgaggccagaggcttgtcgccctgctgcggggggcgctgtccataccagaggactcgacttcgcctgcgatatttatatatgggcccccctcgccggcacctgcggagtcttgctcctgagccttgtgatcacgctttattgtaaccatcggaatagatccaaaagaagccgcctgctccatagcgattacatgaatatgactccacgccgccctggccccacaaggaaacactaccagccttacgcaccacctagagatttcgctgcctatcggagcagggtgaagttttccagatctgcagatgcaccagcgtatcagcagggccagaaccaactgtataacgagctcaacctgggacgcagggaagagtatgacgttttggacaagcgcagaggacgggaccctgagatgggtggcaaaccaagacgaaaaaacccccaggagggtctctataatgagctgcagaaggataagatggctgaagcctattctgaaataggcatgaaaggagagcggagaaggggaaaagggcacgacggtttgtaccagggactcagcactgctacgaaggatacttatgacgctctccacatgcaagccctgccacctaggtaa

SEQ ID NO: 68 - protein, 517 aa, synthetic construct
  REGION 1..517: note = Description of Artificial Sequence: Syntheticpolypeptide
MALPVTALLLPLALLLHAARPQVQLQESGPGLVKPSQTLSLTCTVSGGSISSGGFYWSWIRQHPGKGLEWIGYIHHSGSTHYNPSLKSRVTISIDTSKNLFSLRLSSVTAADTAVYYCASLVYCGGDCYSGFDYWGQGTLVTVSSGGGGSGGGGSGGGGSDIQLTQSPSSLSASVGDRVSFTCQASQDINNFLNWYQQKPGKAPKLLIYDASNLETGVPSRFSGSGSGTDFTFTISSLQPEDIATYYCQQYGNLPFTFGGGTKVEIKRAAALSNSIMYFSHFVPVFLPAKPTTTPAPRPPTPAPTIASQPLSLRPEACRPAAGGAVHTRGLDFACDIYIWAPLAGTCGVLLLSLVITLYCNHRNRSKRSRLLHSDYMNMTPRRPGPTRKHYQPYAPPRDFAAYRSRVKFSRSADAPAYQQGQNQLYNELNLGRREEYDVLDKRRGRDPEMGGKPRRKNPQEGLYNELQKDKMAEAYSEIGMKGERRRGKGHDGLYQGLSTATKDTYDALHMQALPPR

SEQ ID NO: 69 - DNA, 1488 bp, synthetic construct
  misc_feature 1..1488: note = Description of Artificial Sequence: Syntheticpolynucleotide
  source 1..1488: mol_type = other DNA
caggtgcagttgcaggaaagcgggcctggccttgtgaaaccaagccagacactgagcctgacatgcactgtgtccggcgggtccatatcttccgggggtttttattggtcctggatacgccagcatcccgggaaaggacttgaatggattggatatatccaccattccggaagcacccactacaatccaagccttaaatcccgggtgacaatctccatcgacacctcaaagaatcttttttccctgcggttgtcttcagtaactgccgccgataccgctgtgtactactgtgccagcctcgtctattgcggcggagattgttattctgggttcgattattggggtcaaggcacactggtaactgtcagcagcggaggcggcggttccgggggcgggggcagtggagggggcggatctgacattcagcttacgcagtccccatcttcacttagcgccagcgttggcgatcgggtcagcttcacgtgtcaagcaagtcaggatatcaacaactttcttaactggtaccagcagaagccaggcaaggcacccaagttgctgatttacgatgcttctaacctcgagacgggagtgcctagccgcttctccgggagcggcagcggcacagactttacctttacgatttccagtctgcagccagaggatatagcaacttattactgtcagcagtatggcaacctcccttttaccttcggtggtggcacaaaggtcgagattaaaagagccgcagcgttgtccaactccataatgtatttttctcattttgtgcccgtctttctgcctgccaaacctaccaccacccccgccccacgaccacctactccagcccccaccatcgcctcccagcccctcagcctgaggccagaggcttgtcgccctgctgcggggggcgctgtccataccagaggactcgacttcgcctgcgatatttatatatgggcccccctcgccggcacctgcggagtcttgctcctgagccttgtgatcacgctttattgtaaccatcggaatagatccaaaagaagccgcctgctccatagcgattacatgaatatgactccacgccgccctggccccacaaggaaacactaccagccttacgcaccacctagagatttcgctgcctatcggagcagggtgaagttttccagatctgcagatgcaccagcgtatcagcagggccagaaccaactgtataacgagctcaacctgggacgcagggaagagtatgacgttttggacaagcgcagaggacgggaccctgagatgggtggcaaaccaagacgaaaaaacccccaggagggtctctataatgagctgcagaaggataagatggctgaagcctattctgaaataggcatgaaaggagagcggagaaggggaaaagggcacgacggtttgtaccagggactcagcactgctacgaaggatacttatgacgctctccacatgcaagccctgccacctagg

SEQ ID NO: 70 - protein, 496 aa, synthetic construct
  REGION 1..496: note = Description of Artificial Sequence: Syntheticpolypeptide
QVQLQESGPGLVKPSQTLSLTCTVSGGSISSGGFYWSWIRQHPGKGLEWIGYIHHSGSTHYNPSLKSRVTISIDTSKNLFSLRLSSVTAADTAVYYCASLVYCGGDCYSGFDYWGQGTLVTVSSGGGGSGGGGSGGGGSDIQLTQSPSSLSASVGDRVSFTCQASQDINNFLNWYQQKPGKAPKLLIYDASNLETGVPSRFSGSGSGTDFTFTISSLQPEDIATYYCQQYGNLPFTFGGGTKVEIKRAAALSNSIMYFSHFVPVFLPAKPTTTPAPRPPTPAPTIASQPLSLRPEACRPAAGGAVHTRGLDFACDIYIWAPLAGTCGVLLLSLVITLYCNHRNRSKRSRLLHSDYMNMTPRRPGPTRKHYQPYAPPRDFAAYRSRVKFSRSADAPAYQQGQNQLYNELNLGRREEYDVLDKRRGRDPEMGGKPRRKNPQEGLYNELQKDKMAEAYSEIGMKGERRRGKGHDGLYQGLSTATKDTYDALHMQALPPR

SEQ ID NO: 71 - DNA, 363 bp, synthetic construct
  misc_feature 1..363: note = Description of Artificial Sequence: Syntheticpolynucleotide
  source 1..363: mol_type = other DNA
caggtccaactggtgcagtccggagccgaagtcaagaaaccaggtgcctccgttaaagtgagttgcaaagtctctggatacactctgaccgagctctctatgcactgggtccggcaggcccccggcaagggattggaatggatgggcgggttcgatcctgaggacggagagactatctacgctcaaaaattccagggacgagtgactgtgaccgaagacactagtaccgacactgcctacatggaactttcctctctgcgatcagaagataccgcagtgtactactgtgctactgaatctaggggcattggatggccctacttcgattactggggtcagggaactctggtgactgtctccagc

SEQ ID NO: 72 - protein, 121 aa, synthetic construct
  REGION 1..121: note = Description of Artificial Sequence: Syntheticpolypeptide
QVQLVQSGAEVKKPGASVKVSCKVSGYTLTELSMHWVRQAPGKGLEWMGGFDPEDGETIYAQKFQGRVTVTEDTSTDTAYMELSSLRSEDTAVYYCATESRGIGWPYFDYWGQGTLVTVSS

SEQ ID NO: 73 - protein, 7 aa, synthetic construct
  REGION 1..7: note = Description of Artificial Sequence: Syntheticpeptide
GYTLTEL

SEQ ID NO: 74 - protein, 6 aa, synthetic construct
  REGION 1..6: note = Description of Artificial Sequence: Syntheticpeptide
DPEDGE

SEQ ID NO: 75 - protein, 12 aa, synthetic construct
  REGION 1..12: note = Description of Artificial Sequence: Syntheticpeptide
ESRGIGWPYFDY

SEQ ID NO: 76 - DNA, 324 bp, synthetic construct
  misc_feature 1..324: note = Description of Artificial Sequence: Syntheticpolynucleotide
  source 1..324: mol_type = other DNA
gatattcagatgactcaatctccttcttctctgtccgcttccgtgggcgatagagtgaccattacttgtagggcgtcccagtcaatctccagttatttgaattggtatcagcagaagcccgggaaagcacctaagctgttgatcagcggggcttctagcctgaagagtggggtaccttcacggttcagcggaagcggaagcggaaccgatttcaccctgactatcagcagcctgccacctgaggactttgcaacttactactgccaacagtcatacagcactccgatcactttcggccagggcacccggctcgaaatcaagcgc

SEQ ID NO: 77 - protein, 108 aa, synthetic construct
  REGION 1..108: note = Description of Artificial Sequence: Syntheticpolypeptide
DIQMTQSPSSLSASVGDRVTITCRASQSISSYLNWYQQKPGKAPKLLISGASSLKSGVPSRFSGSGSGTDFTLTISSLPPEDFATYYCQQSYSTPITFGQGTRLEIKR

SEQ ID NO: 78 - protein, 11 aa, synthetic construct
  REGION 1..11: note = Description of Artificial Sequence: Syntheticpeptide
RASQSISSYLN

SEQ ID NO: 79 - protein, 7 aa, synthetic construct
  REGION 1..7: note = Description of Artificial Sequence: Syntheticpeptide
GASSLKS

SEQ ID NO: 80 - protein, 9 aa, synthetic construct
  REGION 1..9: note = Description of Artificial Sequence: Syntheticpeptide
QQSYSTPIT

SEQ ID NO: 81 - DNA, 1437 bp, synthetic construct
  misc_feature 1..1437: note = Description of Artificial Sequence: Syntheticpolynucleotide
  source 1..1437: mol_type = other DNA
atggcactccccgtaactgctctgctgctgccgttggcattgctcctgcacgccgcacgcccgcaggtccaactggtgcagtccggagccgaagtcaagaaaccaggtgcctccgttaaagtgagttgcaaagtctctggatacactctgaccgagctctctatgcactgggtccggcaggcccccggcaagggattggaatggatgggcgggttcgatcctgaggacggagagactatctacgctcaaaaattccagggacgagtgactgtgaccgaagacactagtaccgacactgcctacatggaactttcctctctgcgatcagaagataccgcagtgtactactgtgctactgaatctaggggcattggatggccctacttcgattactggggtcagggaactctggtgactgtctccagcggtggaggtggcagcggtggtggcggaagcggggggggcggctctgatattcagatgactcaatctccttcttctctgtccgcttccgtgggcgatagagtgaccattacttgtagggcgtcccagtcaatctccagttatttgaattggtatcagcagaagcccgggaaagcacctaagctgttgatcagcggggcttctagcctgaagagtggggtaccttcacggttcagcggaagcggaagcggaaccgatttcaccctgactatcagcagcctgccacctgaggactttgcaacttactactgccaacagtcatacagcactccgatcactttcggccagggcacccggctcgaaatcaagcgcgctgctgctttggacaatgagaagtcaaacggcaccatcatacatgttaaaggtaaacatctgtgtccctccccgctgttccccggcccttccaaaccgttctgggttctggtggtggtcggaggcgtactcgcttgctatagtctgctggtaactgtcgccttcatcatcttttgggtgagatccaaaagaagccgcctgctccatagcgattacatgaatatgactccacgccgccctggccccacaaggaaacactaccagccttacgcaccacctagagatttcgctgcctatcggagcagggtgaagttttccagatctgcagatgcaccagcgtatcagcagggccagaaccaactgtataacgagctcaacctgggacgcagggaagagtatgacgttttggacaagcgcagaggacgggaccctgagatgggtggcaaaccaagacgaaaaaacccccaggagggtctctataatgagctgcagaaggataagatggctgaagcctattctgaaataggcatgaaaggagagcggagaaggggaaaagggcacgacggtttgtaccagggactcagcactgctacgaaggatacttatgacgctctccacatgcaagccctgccacctaggtaa

SEQ ID NO: 82 - protein, 478 aa, synthetic construct
  REGION 1..478: note = Description of Artificial Sequence: Syntheticpolypeptide
MALPVTALLLPLALLLHAARPQVQLVQSGAEVKKPGASVKVSCKVSGYTLTELSMHWVRQAPGKGLEWMGGFDPEDGETIYAQKFQGRVTVTEDTSTDTAYMELSSLRSEDTAVYYCATESRGIGWPYFDYWGQGTLVTVSSGGGGSGGGGSGGGGSDIQMTQSPSSLSASVGDRVTITCRASQSISSYLNWYQQKPGKAPKLLISGASSLKSGVPSRFSGSGSGTDFTLTISSLPPEDFATYYCQQSYSTPITFGQGTRLEIKRAAALDNEKSNGTIIHVKGKHLCPSPLFPGPSKPFWVLVVVGGVLACYSLLVTVAFIIFWVRSKRSRLLHSDYMNMTPRRPGPTRKHYQPYAPPRDFAAYRSRVKFSRSADAPAYQQGQNQLYNELNLGRREEYDVLDKRRGRDPEMGGKPRRKNPQEGLYNELQKDKMAEAYSEIGMKGERRRGKGHDGLYQGLSTATKDTYDALHMQALPPR

SEQ ID NO: 83 - DNA, 1371 bp, synthetic construct
  misc_feature 1..1371: note = Description of Artificial Sequence: Syntheticpolynucleotide
  source 1..1371: mol_type = other DNA
caggtccaactggtgcagtccggagccgaagtcaagaaaccaggtgcctccgttaaagtgagttgcaaagtctctggatacactctgaccgagctctctatgcactgggtccggcaggcccccggcaagggattggaatggatgggcgggttcgatcctgaggacggagagactatctacgctcaaaaattccagggacgagtgactgtgaccgaagacactagtaccgacactgcctacatggaactttcctctctgcgatcagaagataccgcagtgtactactgtgctactgaatctaggggcattggatggccctacttcgattactggggtcagggaactctggtgactgtctccagcggtggaggtggcagcggtggtggcggaagcggggggggcggctctgatattcagatgactcaatctccttcttctctgtccgcttccgtgggcgatagagtgaccattacttgtagggcgtcccagtcaatctccagttatttgaattggtatcagcagaagcccgggaaagcacctaagctgttgatcagcggggcttctagcctgaagagtggggtaccttcacggttcagcggaagcggaagcggaaccgatttcaccctgactatcagcagcctgccacctgaggactttgcaacttactactgccaacagtcatacagcactccgatcactttcggccagggcacccggctcgaaatcaagcgcgctgctgctttggacaatgagaagtcaaacggcaccatcatacatgttaaaggtaaacatctgtgtccctccccgctgttccccggcccttccaaaccgttctgggttctggtggtggtcggaggcgtactcgcttgctatagtctgctggtaactgtcgccttcatcatcttttgggtgagatccaaaagaagccgcctgctccatagcgattacatgaatatgactccacgccgccctggccccacaaggaaacactaccagccttacgcaccacctagagatttcgctgcctatcggagcagggtgaagttttccagatctgcagatgcaccagcgtatcagcagggccagaaccaactgtataacgagctcaacctgggacgcagggaagagtatgacgttttggacaagcgcagaggacgggaccctgagatgggtggcaaaccaagacgaaaaaacccccaggagggtctctataatgagctgcagaaggataagatggctgaagcctattctgaaataggcatgaaaggagagcggagaaggggaaaagggcacgacggtttgtaccagggactcagcactgctacgaaggatacttatgacgctctccacatgcaagccctgccacctagg

SEQ ID NO: 84 - protein, 457 aa, synthetic construct
  REGION 1..457: note = Description of Artificial Sequence: Syntheticpolypeptide
QVQLVQSGAEVKKPGASVKVSCKVSGYTLTELSMHWVRQAPGKGLEWMGGFDPEDGETIYAQKFQGRVTVTEDTSTDTAYMELSSLRSEDTAVYYCATESRGIGWPYFDYWGQGTLVTVSSGGGGSGGGGSGGGGSDIQMTQSPSSLSASVGDRVTITCRASQSISSYLNWYQQKPGKAPKLLISGASSLKSGVPSRFSGSGSGTDFTLTISSLPPEDFATYYCQQSYSTPITFGQGTRLEIKRAAALDNEKSNGTIIHVKGKHLCPSPLFPGPSKPFWVLVVVGGVLACYSLLVTVAFIIFWVRSKRSRLLHSDYMNMTPRRPGPTRKHYQPYAPPRDFAAYRSRVKFSRSADAPAYQQGQNQLYNELNLGRREEYDVLDKRRGRDPEMGGKPRRKNPQEGLYNELQKDKMAEAYSEIGMKGERRRGKGHDGLYQGLSTATKDTYDALHMQALPPR

SEQ ID NO: 85 - DNA, 1464 bp, synthetic construct
  misc_feature 1..1464: note = Description of Artificial Sequence: Syntheticpolynucleotide
  source 1..1464: mol_type = other DNA
atggcactccccgtaactgctctgctgctgccgttggcattgctcctgcacgccgcacgcccgcaggtgcagcttgtgcagagcggggccgaggtgaagaagcccggggccagcgtcaaagtgtcctgtaaggtcagcggttacaccctcaccgagctgagcatgcactgggtacggcaggctcccggcaaaggtcttgagtggatgggtggatttgatccagaagatggagagactatctacgcccagaagttccagggccgggtcaccgtaacagaagacacctcaactgacaccgcttacatggagctgagttcactgcggtccgaggacacggccgtgtattattgtgccaccgagagccgcggaatcggatggccttacttcgactactggggacagggtacacttgttacagtatcatccgggggtggcggctctggtgggggcggctccggagggggtggatcagatatccaaatgactcaaagtccaagttccctgtctgcctcagtcggagatagagtcaccataacctgcagggcaagtcagtccatctcctcctatctgaactggtaccaacagaaacctggaaaggcgcctaagctcctgatctccggagcctcatctttgaaatccggtgtcccatctcgcttcagtggctctggaagcggtacagattttactttgaccattagcagcctcccaccggaagactttgctacatattactgccagcagtcttactcaaccccaatcaccttcgggcaaggcaccagactcgaaataaaaagagcagctgctatcgaggttatgtacccaccgccgtacttggataacgaaaaaagcaatgggaccatcattcatgtgaagggtaagcacctttgccctagcccactgtttcctggcccgagtaaacccttttgggtacttgtggtcgtcggcggcgtgctggcctgctactcactcctggttaccgtcgcattcatcatcttttgggtgagatccaaaagaagccgcctgctccatagcgattacatgaatatgactccacgccgccctggccccacaaggaaacactaccagccttacgcaccacctagagatttcgctgcctatcggagcagggtgaagttttccagatctgcagatgcaccagcgtatcagcagggccagaaccaactgtataacgagctcaacctgggacgcagggaagagtatgacgttttggacaagcgcagaggacgggaccctgagatgggtggcaaaccaagacgaaaaaacccccaggagggtctctataatgagctgcagaaggataagatggctgaagcctattctgaaataggcatgaaaggagagcggagaaggggaaaagggcacgacggtttgtaccagggactcagcactgctacgaaggatacttatgacgctctccacatgcaagccctgccacctaggtaa

SEQ ID NO: 86 - protein, 487 aa, synthetic construct
  REGION 1..487: note = Description of Artificial Sequence: Syntheticpolypeptide
MALPVTALLLPLALLLHAARPQVQLVQSGAEVKKPGASVKVSCKVSGYTLTELSMHWVRQAPGKGLEWMGGFDPEDGETIYAQKFQGRVTVTEDTSTDTAYMELSSLRSEDTAVYYCATESRGIGWPYFDYWGQGTLVTVSSGGGGSGGGGSGGGGSDIQMTQSPSSLSASVGDRVTITCRASQSISSYLNWYQQKPGKAPKLLISGASSLKSGVPSRFSGSGSGTDFTLTISSLPPEDFATYYCQQSYSTPITFGQGTRLEIKRAAAIEVMYPPPYLDNEKSNGTIIHVKGKHLCPSPLFPGPSKPFWVLVVVGGVLACYSLLVTVAFIIFWVRSKRSRLLHSDYMNMTPRRPGPTRKHYQPYAPPRDFAAYRSRVKFSRSADAPAYQQGQNQLYNELNLGRREEYDVLDKRRGRDPEMGGKPRRKNPQEGLYNELQKDKMAEAYSEIGMKGERRRGKGHDGLYQGLSTATKDTYDALHMQALPPR

SEQ ID NO: 87 - DNA, 1398 bp, synthetic construct
  misc_feature 1..1398: note = Description of Artificial Sequence: Syntheticpolynucleotide
  source 1..1398: mol_type = other DNA
caggtgcagcttgtgcagagcggggccgaggtgaagaagcccggggccagcgtcaaagtgtcctgtaaggtcagcggttacaccctcaccgagctgagcatgcactgggtacggcaggctcccggcaaaggtcttgagtggatgggtggatttgatccagaagatggagagactatctacgcccagaagttccagggccgggtcaccgtaacagaagacacctcaactgacaccgcttacatggagctgagttcactgcggtccgaggacacggccgtgtattattgtgccaccgagagccgcggaatcggatggccttacttcgactactggggacagggtacacttgttacagtatcatccgggggtggcggctctggtgggggcggctccggagggggtggatcagatatccaaatgactcaaagtccaagttccctgtctgcctcagtcggagatagagtcaccataacctgcagggcaagtcagtccatctcctcctatctgaactggtaccaacagaaacctggaaaggcgcctaagctcctgatctccggagcctcatctttgaaatccggtgtcccatctcgcttcagtggctctggaagcggtacagattttactttgaccattagcagcctcccaccggaagactttgctacatattactgccagcagtcttactcaaccccaatcaccttcgggcaaggcaccagactcgaaataaaaagagcagctgctatcgaggttatgtacccaccgccgtacttggataacgaaaaaagcaatgggaccatcattcatgtgaagggtaagcacctttgccctagcccactgtttcctggcccgagtaaacccttttgggtacttgtggtcgtcggcggcgtgctggcctgctactcactcctggttaccgtcgcattcatcatcttttgggtgagatccaaaagaagccgcctgctccatagcgattacatgaatatgactccacgccgccctggccccacaaggaaacactaccagccttacgcaccacctagagatttcgctgcctatcggagcagggtgaagttttccagatctgcagatgcaccagcgtatcagcagggccagaaccaactgtataacgagctcaacctgggacgcagggaagagtatgacgttttggacaagcgcagaggacgggaccctgagatgggtggcaaaccaagacgaaaaaacccccaggagggtctctataatgagctgcagaaggataagatggctgaagcctattctgaaataggcatgaaaggagagcggagaaggggaaaagggcacgacggtttgtaccagggactcagcactgctacgaaggatacttatgacgctctccacatgcaagccctgccacctagg

SEQ ID NO: 88 - protein, 466 aa, synthetic construct
  REGION 1..466: note = Description of Artificial Sequence: Syntheticpolypeptide
QVQLVQSGAEVKKPGASVKVSCKVSGYTLTELSMHWVRQAPGKGLEWMGGFDPEDGETIYAQKFQGRVTVTEDTSTDTAYMELSSLRSEDTAVYYCATESRGIGWPYFDYWGQGTLVTVSSGGGGSGGGGSGGGGSDIQMTQSPSSLSASVGDRVTITCRASQSISSYLNWYQQKPGKAPKLLISGASSLKSGVPSRFSGSGSGTDFTLTISSLPPEDFATYYCQQSYSTPITFGQGTRLEIKRAAAIEVMYPPPYLDNEKSNGTIIHVKGKHLCPSPLFPGPSKPFWVLVVVGGVLACYSLLVTVAFIIFWVRSKRSRLLHSDYMNMTPRRPGPTRKHYQPYAPPRDFAAYRSRVKFSRSADAPAYQQGQNQLYNELNLGRREEYDVLDKRRGRDPEMGGKPRRKNPQEGLYNELQKDKMAEAYSEIGMKGERRRGKGHDGLYQGLSTATKDTYDALHMQALPPR

SEQ ID NO: 89 - DNA, 1545 bp, synthetic construct
  misc_feature 1..1545: note = Description of Artificial Sequence: Syntheticpolynucleotide
  source 1..1545: mol_type = other DNA
atggcactccccgtaactgctctgctgctgccgttggcattgctcctgcacgccgcacgcccgcaggtgcagttggtgcaaagcggcgcagaagttaagaaacctggggcgtcagttaaggtgtcttgcaaagtatctggctataccctcactgagctgtccatgcattgggtaaggcaggctcctggaaaggggctcgaatggatgggaggatttgaccctgaagacggagagaccatctacgcccagaaattccagggtagagtaacagtgactgaggacactagcactgacacagcgtacatggagctgagttctctgagaagtgaggacacagccgtttactactgcgctaccgagtccagaggtattggctggccatacttcgactattggggtcagggcaccctggttacagtgagttcaggaggcgggggctctggggggggcggttccggaggggggggctcagatatacagatgacgcagagtccatcaagtctctcagccagcgtgggagatcgcgtgactattacttgccgcgccagccagagtattagctcctatctgaattggtaccagcaaaagcccgggaaggcccctaagcttctgatttctggcgcctcctctttgaagtcaggtgtgccaagcagatttagcgggtctggaagtggcactgactttacacttactatctccagcctgcccccagaggattttgccacatattactgtcagcaaagctactctactccaatcactttcggccagggcacaagattggagattaagagggctgccgcactttcaaattccatcatgtatttcagccattttgtgcctgtttttcttccggccaaacctacaaccactcccgccccacgcccacctactcccgcccctaccattgcctcccagcctctgtctcttagacctgaggcttgtagacctgctgccggcggagccgtgcacactcgcggtctggacttcgcctgcgacatctatatctgggcccctctggccggcacctgcggcgttctccttctctcactcgtaatcacactctattgcaatcacaggaacagatccaaaagaagccgcctgctccatagcgattacatgaatatgactccacgccgccctggccccacaaggaaacactaccagccttacgcaccacctagagatttcgctgcctatcggagcagggtgaagttttccagatctgcagatgcaccagcgtatcagcagggccagaaccaactgtataacgagctcaacctgggacgcagggaagagtatgacgttttggacaagcgcagaggacgggaccctgagatgggtggcaaaccaagacgaaaaaacccccaggagggtctctataatgagctgcagaaggataagatggctgaagcctattctgaaataggcatgaaaggagagcggagaaggggaaaagggcacgacggtttgtaccagggactcagcactgctacgaaggatacttatgacgctctccacatgcaagccctgccacctaggtaa

SEQ ID NO: 90 - protein, 514 aa, synthetic construct
  REGION 1..514: note = Description of Artificial Sequence: Syntheticpolypeptide
MALPVTALLLPLALLLHAARPQVQLVQSGAEVKKPGASVKVSCKVSGYTLTELSMHWVRQAPGKGLEWMGGFDPEDGETIYAQKFQGRVTVTEDTSTDTAYMELSSLRSEDTAVYYCATESRGIGWPYFDYWGQGTLVTVSSGGGGSGGGGSGGGGSDIQMTQSPSSLSASVGDRVTITCRASQSISSYLNWYQQKPGKAPKLLISGASSLKSGVPSRFSGSGSGTDFTLTISSLPPEDFATYYCQQSYSTPITFGQGTRLEIKRAAALSNSIMYFSHFVPVFLPAKPTTTPAPRPPTPAPTIASQPLSLRPEACRPAAGGAVHTRGLDFACDIYIWAPLAGTCGVLLLSLVITLYCNHRNRSKRSRLLHSDYMNMTPRRPGPTRKHYQPYAPPRDFAAYRSRVKFSRSADAPAYQQGQNQLYNELNLGRREEYDVLDKRRGRDPEMGGKPRRKNPQEGLYNELQKDKMAEAYSEIGMKGERRRGKGHDGLYQGLSTATKDTYDALHMQALPPR

SEQ ID NO: 91 - DNA, 1479 bp, synthetic construct
  misc_feature 1..1479: note = Description of Artificial Sequence: Syntheticpolynucleotide
  source 1..1479: mol_type = other DNA
caggtgcagttggtgcaaagcggcgcagaagttaagaaacctggggcgtcagttaaggtgtcttgcaaagtatctggctataccctcactgagctgtccatgcattgggtaaggcaggctcctggaaaggggctcgaatggatgggaggatttgaccctgaagacggagagaccatctacgcccagaaattccagggtagagtaacagtgactgaggacactagcactgacacagcgtacatggagctgagttctctgagaagtgaggacacagccgtttactactgcgctaccgagtccagaggtattggctggccatacttcgactattggggtcagggcaccctggttacagtgagttcaggaggcgggggctctggggggggcggttccggaggggggggctcagatatacagatgacgcagagtccatcaagtctctcagccagcgtgggagatcgcgtgactattacttgccgcgccagccagagtattagctcctatctgaattggtaccagcaaaagcccgggaaggcccctaagcttctgatttctggcgcctcctctttgaagtcaggtgtgccaagcagatttagcgggtctggaagtggcactgactttacacttactatctccagcctgcccccagaggattttgccacatattactgtcagcaaagctactctactccaatcactttcggccagggcacaagattggagattaagagggctgccgcactttcaaattccatcatgtatttcagccattttgtgcctgtttttcttccggccaaacctacaaccactcccgccccacgcccacctactcccgcccctaccattgcctcccagcctctgtctcttagacctgaggcttgtagacctgctgccggcggagccgtgcacactcgcggtctggacttcgcctgcgacatctatatctgggcccctctggccggcacctgcggcgttctccttctctcactcgtaatcacactctattgcaatcacaggaacagatccaaaagaagccgcctgctccatagcgattacatgaatatgactccacgccgccctggccccacaaggaaacactaccagccttacgcaccacctagagatttcgctgcctatcggagcagggtgaagttttccagatctgcagatgcaccagcgtatcagcagggccagaaccaactgtataacgagctcaacctgggacgcagggaagagtatgacgttttggacaagcgcagaggacgggaccctgagatgggtggcaaaccaagacgaaaaaacccccaggagggtctctataatgagctgcagaaggataagatggctgaagcctattctgaaataggcatgaaaggagagcggagaaggggaaaagggcacgacggtttgtaccagggactcagcactgctacgaaggatacttatgacgctctccacatgcaagccctgccacctagg

SEQ ID NO: 92 - protein, 493 aa, synthetic construct
  REGION 1..493: note = Description of Artificial Sequence: Syntheticpolypeptide
QVQLVQSGAEVKKPGASVKVSCKVSGYTLTELSMHWVRQAPGKGLEWMGGFDPEDGETIYAQKFQGRVTVTEDTSTDTAYMELSSLRSEDTAVYYCATESRGIGWPYFDYWGQGTLVTVSSGGGGSGGGGSGGGGSDIQMTQSPSSLSASVGDRVTITCRASQSISSYLNWYQQKPGKAPKLLISGASSLKSGVPSRFSGSGSGTDFTLTISSLPPEDFATYYCQQSYSTPITFGQGTRLEIKRAAALSNSIMYFSHFVPVFLPAKPTTTPAPRPPTPAPTIASQPLSLRPEACRPAAGGAVHTRGLDFACDIYIWAPLAGTCGVLLLSLVITLYCNHRNRSKRSRLLHSDYMNMTPRRPGPTRKHYQPYAPPRDFAAYRSRVKFSRSADAPAYQQGQNQLYNELNLGRREEYDVLDKRRGRDPEMGGKPRRKNPQEGLYNELQKDKMAEAYSEIGMKGERRRGKGHDGLYQGLSTATKDTYDALHMQALPPR

SEQ ID NO: 93 - DNA, 351 bp, synthetic construct
  misc_feature 1..351: note = Description of Artificial Sequence: Syntheticpolynucleotide
  source 1..351: mol_type = other DNA
caggtccagttggtcgaaagtggcggtggtgtagtgcagccgggccgcagtttgaggctttcctgtgcggcttcaggctttactttttccagctatggaatgcactgggtgcggcaggcccccggcaaaggacttgagtgggtggccgtcatttcttatgacggatcagataagtactacgtggacagcgtcaagggcagattcaccatctctagggacaacagtaaaaatagactctacctccagatgaatagcctcagagctgaagacacggccgtctactattgtgctcgggagcggtatagtggcagagactactgggggcagggcacactcgttacagtgagtagc

SEQ ID NO: 94 - protein, 117 aa, synthetic construct
  REGION 1..117: note = Description of Artificial Sequence: Syntheticpolypeptide
QVQLVESGGGVVQPGRSLRLSCAASGFTFSSYGMHWVRQAPGKGLEWVAVISYDGSDKYYVDSVKGRFTISRDNSKNRLYLQMNSLRAEDTAVYYCARERYSGRDYWGQGTLVTVSS

SEQ ID NO: 95 - protein, 7 aa, synthetic construct
  REGION 1..7: note = Description of Artificial Sequence: Syntheticpeptide
GFTFSSY

SEQ ID NO: 96 - protein, 6 aa, synthetic construct
  REGION 1..6: note = Description of Artificial Sequence: Syntheticpeptide
SYDGSD

SEQ ID NO: 97 - protein, 8 aa, synthetic construct
  REGION 1..8: note = Description of Artificial Sequence: Syntheticpeptide
ERYSGRDY

SEQ ID NO: 98 - DNA, 324 bp, synthetic construct
  misc_feature 1..324: note = Description of Artificial Sequence: Syntheticpolynucleotide
  source 1..324: mol_type = other DNA
gagattgttatgacccagagtcctgcgaccctctcagtcagccccggggagcgcgcaactttgtcttgcagagctagtcagtccgtgtcctctcttctgacatggtaccagcaaaagcccgggcaggctccgcgccttttgatctttggggcttcaacaagagccactgggattcccgcacgattctctggctccgggagcggtactggtttcaccctgacgattagcagtctccagagcgaggacttcgccgtatactactgccagcagtacgatacgtggccattcacttttggaccagggactaaagtggattttaagcgc

SEQ ID NO: 99 - protein, 108 aa, synthetic construct
  REGION 1..108: note = Description of Artificial Sequence: Syntheticpolypeptide
EIVMTQSPATLSVSPGERATLSCRASQSVSSLLTWYQQKPGQAPRLLIFGASTRATGIPARFSGSGSGTGFTLTISSLQSEDFAVYYCQQYDTWPFTFGPGTKVDFKR

SEQ ID NO: 100 - protein, 11 aa, synthetic construct
  REGION 1..11: note = Description of Artificial Sequence: Syntheticpeptide
RASQSVSSLLT

SEQ ID NO: 101 - protein, 7 aa, synthetic construct
  REGION 1..7: note = Description of Artificial Sequence: Syntheticpeptide
GASTRAT

SEQ ID NO: 102 - protein, 9 aa, synthetic construct
  REGION 1..9: note = Description of Artificial Sequence: Syntheticpeptide
QQYDTWPFT

SEQ ID NO: 103 - DNA, 1425 bp, synthetic construct
  misc_feature 1..1425: note = Description of Artificial Sequence: Syntheticpolynucleotide
  source 1..1425: mol_type = other DNA
atggcactccccgtaactgctctgctgctgccgttggcattgctcctgcacgccgcacgcccgcaggtccagttggtcgaaagtggcggtggtgtagtgcagccgggccgcagtttgaggctttcctgtgcggcttcaggctttactttttccagctatggaatgcactgggtgcggcaggcccccggcaaaggacttgagtgggtggccgtcatttcttatgacggatcagataagtactacgtggacagcgtcaagggcagattcaccatctctagggacaacagtaaaaatagactctacctccagatgaatagcctcagagctgaagacacggccgtctactattgtgctcgggagcggtatagtggcagagactactgggggcagggcacactcgttacagtgagtagcggcggaggagggagtgggggcggtggctccggtggaggaggttctgagattgttatgacccagagtcctgcgaccctctcagtcagccccggggagcgcgcaactttgtcttgcagagctagtcagtccgtgtcctctcttctgacatggtaccagcaaaagcccgggcaggctccgcgccttttgatctttggggcttcaacaagagccactgggattcccgcacgattctctggctccgggagcggtactggtttcaccctgacgattagcagtctccagagcgaggacttcgccgtatactactgccagcagtacgatacgtggccattcacttttggaccagggactaaagtggattttaagcgcgccgccgctctcgataacgaaaagtcaaatggcaccataatccacgtcaaaggcaagcacctgtgcccttccccgctcttccccggacccagtaaaccattttgggtgctggttgttgtggggggcgtgctggcctgctatagccttttggtcactgtagccttcattattttttgggtcagatccaaaagaagccgcctgctccatagcgattacatgaatatgactccacgccgccctggccccacaaggaaacactaccagccttacgcaccacctagagatttcgctgcctatcggagcagggtgaagttttccagatctgcagatgcaccagcgtatcagcagggccagaaccaactgtataacgagctcaacctgggacgcagggaagagtatgacgttttggacaagcgcagaggacgggaccctgagatgggtggcaaaccaagacgaaaaaacccccaggagggtctctataatgagctgcagaaggataagatggctgaagcctattctgaaataggcatgaaaggagagcggagaaggggaaaagggcacgacggtttgtaccagggactcagcactgctacgaaggatacttatgacgctctccacatgcaagccctgccacctaggtaa

SEQ ID NO: 104 - protein, 474 aa, synthetic construct
  REGION 1..474: note = Description of Artificial Sequence: Syntheticpolypeptide
MALPVTALLLPLALLLHAARPQVQLVESGGGVVQPGRSLRLSCAASGFTFSSYGMHWVRQAPGKGLEWVAVISYDGSDKYYVDSVKGRFTISRDNSKNRLYLQMNSLRAEDTAVYYCARERYSGRDYWGQGTLVTVSSGGGGSGGGGSGGGGSEIVMTQSPATLSVSPGERATLSCRASQSVSSLLTWYQQKPGQAPRLLIFGASTRATGIPARFSGSGSGTGFTLTISSLQSEDFAVYYCQQYDTWPFTFGPGTKVDFKRAAALDNEKSNGTIIHVKGKHLCPSPLFPGPSKPFWVLVVVGGVLACYSLLVTVAFIIFWVRSKRSRLLHSDYMNMTPRRPGPTRKHYQPYAPPRDFAAYRSRVKFSRSADAPAYQQGQNQLYNELNLGRREEYDVLDKRRGRDPEMGGKPRRKNPQEGLYNELQKDKMAEAYSEIGMKGERRRGKGHDGLYQGLSTATKDTYDALHMQALPPR

SEQ ID NO: 105 - DNA, 1359 bp, synthetic construct
  misc_feature 1..1359: note = Description of Artificial Sequence: Syntheticpolynucleotide
  source 1..1359: mol_type = other DNA
caggtccagttggtcgaaagtggcggtggtgtagtgcagccgggccgcagtttgaggctttcctgtgcggcttcaggctttactttttccagctatggaatgcactgggtgcggcaggcccccggcaaaggacttgagtgggtggccgtcatttcttatgacggatcagataagtactacgtggacagcgtcaagggcagattcaccatctctagggacaacagtaaaaatagactctacctccagatgaatagcctcagagctgaagacacggccgtctactattgtgctcgggagcggtatagtggcagagactactgggggcagggcacactcgttacagtgagtagcggcggaggagggagtgggggcggtggctccggtggaggaggttctgagattgttatgacccagagtcctgcgaccctctcagtcagccccggggagcgcgcaactttgtcttgcagagctagtcagtccgtgtcctctcttctgacatggtaccagcaaaagcccgggcaggctccgcgccttttgatctttggggcttcaacaagagccactgggattcccgcacgattctctggctccgggagcggtactggtttcaccctgacgattagcagtctccagagcgaggacttcgccgtatactactgccagcagtacgatacgtggccattcacttttggaccagggactaaagtggattttaagcgcgccgccgctctcgataacgaaaagtcaaatggcaccataatccacgtcaaaggcaagcacctgtgcccttccccgctcttccccggacccagtaaaccattttgggtgctggttgttgtggggggcgtgctggcctgctatagccttttggtcactgtagccttcattattttttgggtcagatccaaaagaagccgcctgctccatagcgattacatgaatatgactccacgccgccctggccccacaaggaaacactaccagccttacgcaccacctagagatttcgctgcctatcggagcagggtgaagttttccagatctgcagatgcaccagcgtatcagcagggccagaaccaactgtataacgagctcaacctgggacgcagggaagagtatgacgttttggacaagcgcagaggacgggaccctgagatgggtggcaaaccaagacgaaaaaacccccaggagggtctctataatgagctgcagaaggataagatggctgaagcctattctgaaataggcatgaaaggagagcggagaaggggaaaagggcacgacggtttgtaccagggactcagcactgctacgaaggatacttatgacgctctccacatgcaagccctgccacctagg

SEQ ID NO: 106 - protein, 453 aa, synthetic construct
  REGION 1..453: note = Description of Artificial Sequence: Syntheticpolypeptide
QVQLVESGGGVVQPGRSLRLSCAASGFTFSSYGMHWVRQAPGKGLEWVAVISYDGSDKYYVDSVKGRFTISRDNSKNRLYLQMNSLRAEDTAVYYCARERYSGRDYWGQGTLVTVSSGGGGSGGGGSGGGGSEIVMTQSPATLSVSPGERATLSCRASQSVSSLLTWYQQKPGQAPRLLIFGASTRATGIPARFSGSGSGTGFTLTISSLQSEDFAVYYCQQYDTWPFTFGPGTKVDFKRAAALDNEKSNGTIIHVKGKHLCPSPLFPGPSKPFWVLVVVGGVLACYSLLVTVAFIIFWVRSKRSRLLHSDYMNMTPRRPGPTRKHYQPYAPPRDFAAYRSRVKFSRSADAPAYQQGQNQLYNELNLGRREEYDVLDKRRGRDPEMGGKPRRKNPQEGLYNELQKDKMAEAYSEIGMKGERRRGKGHDGLYQGLSTATKDTYDALHMQALPPR

SEQ ID NO: 107 - DNA, 1452 bp, synthetic construct
  misc_feature 1..1452: note = Description of Artificial Sequence: Syntheticpolynucleotide
  source 1..1452: mol_type = other DNA
atggcactccccgtaactgctctgctgctgccgttggcattgctcctgcacgccgcacgcccgcaggtgcagctcgtggagtctggcggcggcgtggtccagcccggccggtccctgcgcctgtcctgcgccgccagcgggtttactttttcctcctacggcatgcactgggtgcgccaggctcccggcaagggcctcgagtgggtcgccgtgatctcatacgatgggtcagacaaatactatgtcgattctgttaaagggcggtttaccatttcaagagataactctaagaataggctgtatttgcagatgaacagcctgagggctgaagataccgcagtgtactattgcgctagggagcggtatagtggccgcgattactggggacagggtacactggtgaccgtgagctctgggggtggcggaagcgggggtggcggaagcggcggagggggtagtgaaattgtgatgacccagtctccggctacactttcagtctcccctggggagagagctacactgtcatgcagagcgtcccagtccgtctcttctctccttacctggtatcagcagaagcccggccaggctcctcgactgctgatcttcggtgcctccacaagggcgaccgggattccagcccgcttctcaggttctgggagcggaactggtttcactttgacaatcagttcactgcagtcagaggatttcgccgtgtactactgccagcaatacgacacatggccattcactttcggacccggtaccaaagtcgatttcaagagagccgcggccatcgaggttatgtacccaccaccatatctggacaatgaaaaaagcaatggaaccattatccatgtgaagggtaaacacctctgccctagcccacttttccctggcccatcaaagcccttctgggtcttggtggtcgtggggggtgtgctggcctgttacagccttctggtgacggttgctttcattatcttctgggttagatccaaaagaagccgcctgctccatagcgattacatgaatatgactccacgccgccctggccccacaaggaaacactaccagccttacgcaccacctagagatttcgctgcctatcggagcagggtgaagttttccagatctgcagatgcaccagcgtatcagcagggccagaaccaactgtataacgagctcaacctgggacgcagggaagagtatgacgttttggacaagcgcagaggacgggaccctgagatgggtggcaaaccaagacgaaaaaacccccaggagggtctctataatgagctgcagaaggataagatggctgaagcctattctgaaataggcatgaaaggagagcggagaaggggaaaagggcacgacggtttgtaccagggactcagcactgctacgaaggatacttatgacgctctccacatgcaagccctgccacctaggtaa

SEQ ID NO: 108 - protein, 483 aa, synthetic construct
  REGION 1..483: note = Description of Artificial Sequence: Syntheticpolypeptide
MALPVTALLLPLALLLHAARPQVQLVESGGGVVQPGRSLRLSCAASGFTFSSYGMHWVRQAPGKGLEWVAVISYDGSDKYYVDSVKGRFTISRDNSKNRLYLQMNSLRAEDTAVYYCARERYSGRDYWGQGTLVTVSSGGGGSGGGGSGGGGSEIVMTQSPATLSVSPGERATLSCRASQSVSSLLTWYQQKPGQAPRLLIFGASTRATGIPARFSGSGSGTGFTLTISSLQSEDFAVYYCQQYDTWPFTFGPGTKVDFKRAAAIEVMYPPPYLDNEKSNGTIIHVKGKHLCPSPLFPGPSKPFWVLVVVGGVLACYSLLVTVAFIIFWVRSKRSRLLHSDYMNMTPRRPGPTRKHYQPYAPPRDFAAYRSRVKFSRSADAPAYQQGQNQLYNELNLGRREEYDVLDKRRGRDPEMGGKPRRKNPQEGLYNELQKDKMAEAYSEIGMKGERRRGKGHDGLYQGLSTATKDTYDALHMQALPPR

SEQ ID NO: 109 - DNA, 1386 bp, synthetic construct
  misc_feature 1..1386: note = Description of Artificial Sequence: Syntheticpolynucleotide
  source 1..1386: mol_type = other DNA
caggtgcagctcgtggagtctggcggcggcgtggtccagcccggccggtccctgcgcctgtcctgcgccgccagcgggtttactttttcctcctacggcatgcactgggtgcgccaggctcccggcaagggcctcgagtgggtcgccgtgatctcatacgatgggtcagacaaatactatgtcgattctgttaaagggcggtttaccatttcaagagataactctaagaataggctgtatttgcagatgaacagcctgagggctgaagataccgcagtgtactattgcgctagggagcggtatagtggccgcgattactggggacagggtacactggtgaccgtgagctctgggggtggcggaagcgggggtggcggaagcggcggagggggtagtgaaattgtgatgacccagtctccggctacactttcagtctcccctggggagagagctacactgtcatgcagagcgtcccagtccgtctcttctctccttacctggtatcagcagaagcccggccaggctcctcgactgctgatcttcggtgcctccacaagggcgaccgggattccagcccgcttctcaggttctgggagcggaactggtttcactttgacaatcagttcactgcagtcagaggatttcgccgtgtactactgccagcaatacgacacatggccattcactttcggacccggtaccaaagtcgatttcaagagagccgcggccatcgaggttatgtacccaccaccatatctggacaatgaaaaaagcaatggaaccattatccatgtgaagggtaaacacctctgccctagcccacttttccctggcccatcaaagcccttctgggtcttggtggtcgtggggggtgtgctggcctgttacagccttctggtgacggttgctttcattatcttctgggttagatccaaaagaagccgcctgctccatagcgattacatgaatatgactccacgccgccctggccccacaaggaaacactaccagccttacgcaccacctagagatttcgctgcctatcggagcagggtgaagttttccagatctgcagatgcaccagcgtatcagcagggccagaaccaactgtataacgagctcaacctgggacgcagggaagagtatgacgttttggacaagcgcagaggacgggaccctgagatgggtggcaaaccaagacgaaaaaacccccaggagggtctctataatgagctgcagaaggataagatggctgaagcctattctgaaataggcatgaaaggagagcggagaaggggaaaagggcacgacggtttgtaccagggactcagcactgctacgaaggatacttatgacgctctccacatgcaagccctgccacctagg

SEQ ID NO: 110 - protein, 462 aa, synthetic construct
  REGION 1..462: note = Description of Artificial Sequence: Syntheticpolypeptide
QVQLVESGGGVVQPGRSLRLSCAASGFTFSSYGMHWVRQAPGKGLEWVAVISYDGSDKYYVDSVKGRFTISRDNSKNRLYLQMNSLRAEDTAVYYCARERYSGRDYWGQGTLVTVSSGGGGSGGGGSGGGGSEIVMTQSPATLSVSPGERATLSCRASQSVSSLLTWYQQKPGQAPRLLIFGASTRATGIPARFSGSGSGTGFTLTISSLQSEDFAVYYCQQYDTWPFTFGPGTKVDFKRAAAIEVMYPPPYLDNEKSNGTIIHVKGKHLCPSPLFPGPSKPFWVLVVVGGVLACYSLLVTVAFIIFWVRSKRSRLLHSDYMNMTPRRPGPTRKHYQPYAPPRDFAAYRSRVKFSRSADAPAYQQGQNQLYNELNLGRREEYDVLDKRRGRDPEMGGKPRRKNPQEGLYNELQKDKMAEAYSEIGMKGERRRGKGHDGLYQGLSTATKDTYDALHMQALPPR

SEQ ID NO: 111 - DNA, 1533 bp, synthetic construct
  misc_feature 1..1533: note = Description of Artificial Sequence: Syntheticpolynucleotide
  source 1..1533: mol_type = other DNA
atggcactccccgtaactgctctgctgctgccgttggcattgctcctgcacgccgcacgcccgcaggtgcagttggttgaatcaggagggggtgtggtgcaacccggtcggtcactgcgcctcagttgtgctgcttccgggtttactttcagctcatatgggatgcactgggtacggcaggctccaggtaaaggcttggaatgggtggcggtgatcagctatgacggctctgacaaatattatgtggactccgtgaaaggcagattcaccatcagtcgagacaactcaaagaatagactctacttgcagatgaatagcctccgggccgaagatactgcagtctattattgcgcccgggagcgctacagtggaagagactattgggggcaaggaactcttgtcacagtctcatctggcggcggcggcagcggtgggggcggatctggcgggggcggcagcgaaatcgttatgactcagagtcctgccacactgagcgttagccctggtgagagagcaacacttagctgcagagctagtcagagtgtttccagtcttttgacatggtaccaacagaagcccggtcaagctccacgactgctcatcttcggtgcatccacccgcgcaaccgggatacccgcccggttttccggttctggaagtggcacaggattcacgctcaccatttcttctctgcagtctgaagactttgccgtgtattactgccagcagtacgatacctggccctttacctttggcccaggtactaaagtggattttaaacgagctgctgcactttccaatagtattatgtacttttcacattttgtgcccgtgttcctgcctgcgaagcctacgacaaccccagcccctaggccgcccacaccggccccaactattgcctcccagccattgtctctgagacccgaagcttgcagacctgctgctggaggcgccgttcacacccgaggattggatttcgcatgtgacatttacatctgggcccctttggccggaacctgcggtgtgctgctgctgtcactcgtgattacactttactgcaaccaccgaaacagatccaaaagaagccgcctgctccatagcgattacatgaatatgactccacgccgccctggccccacaaggaaacactaccagccttacgcaccacctagagatttcgctgcctatcggagcagggtgaagttttccagatctgcagatgcaccagcgtatcagcagggccagaaccaactgtataacgagctcaacctgggacgcagggaagagtatgacgttttggacaagcgcagaggacgggaccctgagatgggtggcaaaccaagacgaaaaaacccccaggagggtctctataatgagctgcagaaggataagatggctgaagcctattctgaaataggcatgaaaggagagcggagaaggggaaaagggcacgacggtttgtaccagggactcagcactgctacgaaggatacttatgacgctctccacatgcaagccctgccacctaggtaa

SEQ ID NO: 112 - protein, 509 aa, synthetic construct
  REGION 1..509: note = Description of Artificial Sequence: Syntheticpolypeptide
MALPVTALLLPLALLLHAARPQVQLVESGGGVVQPGRSLRLSCAASGFTFSSYGMHWVRQAPGKGLEWVAVISYDGSDKYYVDSVKGRFTISRDNSKNRLYLQMNSLRAEDTAVYYCARERYSGRDYWGGTLVTVSSGGGGSGGGGSGGGGSEIVMTQSPATLSVSPGERATLSCRASQSVSSLLTWYQQKPGQAPRLLIFGASTRATGIPARFSGSGSGTGFTLTISSLQSEDFAVYYCQQYDTWPFTFGPGTKVDFKRAAALSNSIMYFSHFVPVFLPAKPTTTPAPRPPTPAPTIASQPLSLRPEACRPAAGGAVHTRGLDFACDIYIWAPLAGTCGVLLLSLVITLYCNHRNRSKRSRLLHSDYMNMTPRRPGPTRKHYQPYAPPRDFAAYRSRVKFSRSADAPAYQQGQNQLYNELNLGRREEYDVLDKRRGRDPEMGGKPRRKNPQEGLYNELQKDKMAEAYSEIGMKGERRRGKGHDGLYQGLSTATKDTYDALHMQALPPR

SEQ ID NO: 113 - DNA, 1467 bp, synthetic construct
  misc_feature 1..1467: note = Description of Artificial Sequence: Syntheticpolynucleotide
  source 1..1467: mol_type = other DNA
caggtgcagttggttgaatcaggagggggtgtggtgcaacccggtcggtcactgcgcctcagttgtgctgcttccgggtttactttcagctcatatgggatgcactgggtacggcaggctccaggtaaaggcttggaatgggtggcggtgatcagctatgacggctctgacaaatattatgtggactccgtgaaaggcagattcaccatcagtcgagacaactcaaagaatagactctacttgcagatgaatagcctccgggccgaagatactgcagtctattattgcgcccgggagcgctacagtggaagagactattgggggcaaggaactcttgtcacagtctcatctggcggcggcggcagcggtgggggcggatctggcgggggcggcagcgaaatcgttatgactcagagtcctgccacactgagcgttagccctggtgagagagcaacacttagctgcagagctagtcagagtgtttccagtcttttgacatggtaccaacagaagcccggtcaagctccacgactgctcatcttcggtgcatccacccgcgcaaccgggatacccgcccggttttccggttctggaagtggcacaggattcacgctcaccatttcttctctgcagtctgaagactttgccgtgtattactgccagcagtacgatacctggccctttacctttggcccaggtactaaagtggattttaaacgagctgctgcactttccaatagtattatgtacttttcacattttgtgcccgtgttcctgcctgcgaagcctacgacaaccccagcccctaggccgcccacaccggccccaactattgcctcccagccattgtctctgagacccgaagcttgcagacctgctgctggaggcgccgttcacacccgaggattggatttcgcatgtgacatttacatctgggcccctttggccggaacctgcggtgtgctgctgctgtcactcgtgattacactttactgcaaccaccgaaacagatccaaaagaagccgcctgctccatagcgattacatgaatatgactccacgccgccctggccccacaaggaaacactaccagccttacgcaccacctagagatttcgctgcctatcggagcagggtgaagttttccagatctgcagatgcaccagcgtatcagcagggccagaaccaactgtataacgagctcaacctgggacgcagggaagagtatgacgttttggacaagcgcagaggacgggaccctgagatgggtggcaaaccaagacgaaaaaacccccaggagggtctctataatgagctgcagaaggataagatggctgaagcctattctgaaataggcatgaaaggagagcggagaaggggaaaagggcacgacggtttgtaccagggactcagcactgctacgaaggatacttatgacgctctccacatgcaagccctgccacctagg

SEQ ID NO: 114 - protein, 489 aa, synthetic construct
  REGION 1..489: note = Description of Artificial Sequence: Syntheticpolypeptide
QVQLVESGGGVVQPGRSLRLSCAASGFTFSSYGMHWVRQAPGKGLEWVAVISYDGSDKYYVDSVKGRFTISRDNSKNRLYLQMNSLRAEDTAVYYCARERYSGRDYWGQGTLVTVSSGGGGSGGGGSGGGGSEIVMTQSPATLSVSPGERATLSCRASQSVSSLLTWYQQKPGQAPRLLIFGASTRATGIPARFSGSGSGTGFTLTISSLQSEDFAVYYCQQYDTWPFTFGPGTKVDFKRAAALSNSIMYFSHFVPVFLPAKPTTTPAPRPPTPAPTIASQPLSLRPEACRPAAGGAVHTRGLDFACDIYIWAPLAGTCGVLLLSLVITLYCNHRNRSKRSRLLHSDYMNMTPRRPGPTRKHYQPYAPPRDFAAYRSRVKFSRSADAPAYQQGQNQLYNELNLGRREEYDVLDKRRGRDPEMGGKPRRKNPQEGLYNELQKDKMAEAYSEIGMKGERRRGKGHDGLYQGLSTATKDTYDALHMQALPPR

SEQ ID NO: 115 - DNA, 1425 bp, synthetic construct
  misc_feature 1..1425: note = Description of Artificial Sequence: Syntheticpolynucleotide
  source 1..1425: mol_type = other DNA
atggcactccccgtaactgctctgctgctgccgttggcattgctcctgcacgccgcacgcccggagattgtgatgacccagtcccctgctaccctgtccgtcagtccgggcgagagagccaccttgtcatgccgggccagccagtccgtcagcagtctcctgacttggtatcagcaaaaaccagggcaggcaccgcggcttttgatttttggtgcaagcacacgcgccactggcattccagctaggttttctggaagtggatctgggacaggcttcactctgacaatcagtagcctgcagagtgaggactttgctgtttactactgtcaacagtacgacacctggccattcacattcgggcccggcaccaaggtcgacttcaagaggggcggtggaggttcaggtggtggcgggtcaggcggcggtgggtctcaggttcaactggtggaatcaggtggcggcgttgtccaaccggggcgatcacttcgactttcctgtgctgcctcaggctttactttttcatcctatgggatgcactgggttcggcaggctcccggaaaaggactcgagtgggttgcagtgatctcttacgatggctcagacaagtattatgtggactcagtcaaggggagattcacaataagccgagacaactccaaaaaccggctttatctccagatgaacagccttagagcggaagataccgcggtatactactgtgcccgcgagaggtattccggcagagactactggggacagggcacactggtcaccgtgagttctgccgcagcgctcgataacgaaaagagcaacggaaccattatccacgttaagggcaagcacctgtgccccagtcccctcttcccaggaccatctaaacccttctgggttctggtagtagttggaggggtccttgcatgttactcccttttggtcaccgtcgccttcattattttctgggtgagatccaaaagaagccgcctgctccatagcgattacatgaatatgactccacgccgccctggccccacaaggaaacactaccagccttacgcaccacctagagatttcgctgcctatcggagcagggtgaagttttccagatctgcagatgcaccagcgtatcagcagggccagaaccaactgtataacgagctcaacctgggacgcagggaagagtatgacgttttggacaagcgcagaggacgggaccctgagatgggtggcaaaccaagacgaaaaaacccccaggagggtctctataatgagctgcagaaggataagatggctgaagcctattctgaaataggcatgaaaggagagcggagaaggggaaaagggcacgacggtttgtaccagggactcagcactgctacgaaggatacttatgacgctctccacatgcaagccctgccacctaggtaa

SEQ ID NO: 116 - protein, 474 aa, synthetic construct
  REGION 1..474: note = Description of Artificial Sequence: Syntheticpolypeptide
MALPVTALLLPLALLLHAARPEIVMTQSPATLSVSPGERATLSCRASQSVSSLLTWYQQKPGQAPRLLIFGASTRATGIPARFSGSGSGTGFTLTISSLQSEDFAVYYCQQYDTWPFTFGPGTKVDFKRGGGGSGGGGSGGGGSQVQLVESGGGVVQPGRSLRLSCAASGFTFSSYGMHWVRQAPGKGLEWVAVISYDGSDKYYVDSVKGRFTISRDNSKNRLYLQMNSLRAEDTAVYYCARERYSGRDYWGQGTLVTVSSAAALDNEKSNGTIIHVKGKHLCPSPLFPGPSKPFWVLVVVGGVLACYSLLVTVAFIIFWVRSKRSRLLHSDYMNMTPRRPGPTRKHYQPYAPPRDFAAYRSRVKFSRSADAPAYQQGQNQLYNELNLGRREEYDVLDKRRGRDPEMGGKPRRKNPQEGLYNELQKDKMAEAYSEIGMKGERRRGKGHDGLYQGLSTATKDTYDALHMQALPPR

SEQ ID NO: 117 - DNA, 1359 bp, synthetic construct
  misc_feature 1..1359: note = Description of Artificial Sequence: Syntheticpolynucleotide
  source 1..1359: mol_type = other DNA
gagattgtgatgacccagtcccctgctaccctgtccgtcagtccgggcgagagagccaccttgtcatgccgggccagccagtccgtcagcagtctcctgacttggtatcagcaaaaaccagggcaggcaccgcggcttttgatttttggtgcaagcacacgcgccactggcattccagctaggttttctggaagtggatctgggacaggcttcactctgacaatcagtagcctgcagagtgaggactttgctgtttactactgtcaacagtacgacacctggccattcacattcgggcccggcaccaaggtcgacttcaagaggggcggtggaggttcaggtggtggcgggtcaggcggcggtgggtctcaggttcaactggtggaatcaggtggcggcgttgtccaaccggggcgatcacttcgactttcctgtgctgcctcaggctttactttttcatcctatgggatgcactgggttcggcaggctcccggaaaaggactcgagtgggttgcagtgatctcttacgatggctcagacaagtattatgtggactcagtcaaggggagattcacaataagccgagacaactccaaaaaccggctttatctccagatgaacagccttagagcggaagataccgcggtatactactgtgcccgcgagaggtattccggcagagactactggggacagggcacactggtcaccgtgagttctgccgcagcgctcgataacgaaaagagcaacggaaccattatccacgttaagggcaagcacctgtgccccagtcccctcttcccaggaccatctaaacccttctgggttctggtagtagttggaggggtccttgcatgttactcccttttggtcaccgtcgccttcattattttctgggtgagatccaaaagaagccgcctgctccatagcgattacatgaatatgactccacgccgccctggccccacaaggaaacactaccagccttacgcaccacctagagatttcgctgcctatcggagcagggtgaagttttccagatctgcagatgcaccagcgtatcagcagggccagaaccaactgtataacgagctcaacctgggacgcagggaagagtatgacgttttggacaagcgcagaggacgggaccctgagatgggtggcaaaccaagacgaaaaaacccccaggagggtctctataatgagctgcagaaggataagatggctgaagcctattctgaaataggcatgaaaggagagcggagaaggggaaaagggcacgacggtttgtaccagggactcagcactgctacgaaggatacttatgacgctctccacatgcaagccctgccacctagg

SEQ ID NO: 118 - protein, 453 aa, synthetic construct
  REGION 1..453: note = Description of Artificial Sequence: Syntheticpolypeptide
EIVMTQSPATLSVSPGERATLSCRASQSVSSLLTWYQQKPGQAPRLLIFGASTRATGIPARFSGSGSGTGFTLTISSLQSEDFAVYYCQQYDTWPFTFGPGTKVDFKRGGGGSGGGGSGGGGSQVQLVESGGGVVQPGRSLRLSCAASGFTFSSYGMHWVRQAPGKGLEWVAVISYDGSDKYYVDSVKGRFTISRDNSKNRLYLQMNSLRAEDTAVYYCARERYSGRDYWGQGTLVTVSSAAALDNEKSNGTIIHVKGKHLCPSPLFPGPSKPFWVLVVVGGVLACYSLLVTVAFIIFWVRSKRSRLLHSDYMNMTPRRPGPTRKHYQPYAPPRDFAAYRSRVKFSRSADAPAYQQGQNQLYNELNLGRREEYDVLDKRRGRDPEMGGKPRRKNPQEGLYNELQKDKMAEAYSEIGMKGERRRGKGHDGLYQGLSTATKDTYDALHMQALPPR

SEQ ID NO: 119 - DNA, 1452 bp, synthetic construct
  misc_feature 1..1452: note = Description of Artificial Sequence: Syntheticpolynucleotide
  source 1..1452: mol_type = other DNA
atggcactccccgtaactgctctgctgctgccgttggcattgctcctgcacgccgcacgcccggagatcgtcatgacacagagtccagctaccctgagcgtgtcccctggagagagagccaccctgtcctgtagggctagtcagagtgtgtccagcctcctcacctggtatcaacagaagcctggtcaagctccccggctgcttatcttcggggccagcacgcgagccacaggcatcccggccagattctctggctctggcagtggcaccgggttcactctcacgatctcatccctgcagtcagaggatttcgctgtgtattactgtcagcagtacgatacatggcccttcaccttcggcccgggcacaaaagtagatttcaagcgcggcggcgggggtagtgggggcgggggatcaggaggagggggctcccaagtacagctggttgagagcggcggcggggtggttcagcccgggcgcagcctcaggctgagttgcgcagcatcaggattcacattcagttcttatggaatgcattgggtcagacaggctcccgggaagggccttgaatgggtggcagtcattagctacgacggaagcgataagtactatgtggactcagttaaagggagatttactatcagccgcgacaattccaaaaacagattgtatttgcagatgaactccctcagggcggaggacactgctgtatattactgcgcacgagagagatactccggccgagactattggggccaaggaacattggtaactgtgagctccgccgcagctattgaggtcatgtaccccccaccttatctcgataatgagaagagtaatgggactataattcacgtaaagggcaaacacctgtgcccttccccgctgtttccaggtccaagtaagccgttctgggtcctggttgtggtgggaggggtgctggcctgctattctctgttggttaccgtggcctttatcattttctgggtgagatccaaaagaagccgcctgctccatagcgattacatgaatatgactccacgccgccctggccccacaaggaaacactaccagccttacgcaccacctagagatttcgctgcctatcggagcagggtgaagttttccagatctgcagatgcaccagcgtatcagcagggccagaaccaactgtataacgagctcaacctgggacgcagggaagagtatgacgttttggacaagcgcagaggacgggaccctgagatgggtggcaaaccaagacgaaaaaacccccaggagggtctctataatgagctgcagaaggataagatggctgaagcctattctgaaataggcatgaaaggagagcggagaaggggaaaagggcacgacggtttgtaccagggactcagcactgctacgaaggatacttatgacgctctccacatgcaagccctgccacctaggtaa

SEQ ID NO: 120 - protein, 483 aa, synthetic construct
  REGION 1..483: note = Description of Artificial Sequence: Syntheticpolypeptide
MALPVTALLLPLALLLHAARPEIVMTQSPATLSVSPGERATLSCRASQSVSSLLTWYQQKPGQAPRLLIFGASTRATGIPARFSGSGSGTGFTLTISSLQSEDFAVYYCQQYDTWPFTFGPGTKVDFKRGGGGSGGGGSGGGGSQVQLVESGGGVVQPGRSLRLSCAASGFTFSSYGMHWVRQAPGKGLEWVAVISYDGSDKYYVDSVKGRFTISRDNSKNRLYLQMNSLRAEDTAVYYCARERYSGRDYWGQGTLVTVSSAAAIEVMYPPPYLDNEKSNGTIIHVKGKHLCPSPLFPGPSKPFWVLVVVGGVLACYSLLVTVAFIIFWVRSKRSRLLHSDYMNMTPRRPGPTRKHYQPYAPPRDFAAYRSRVKFSRSADAPAYQQGQNQLYNELNLGRREEYDVLDKRRGRDPEMGGKPRRKNPQEGLYNELQKDKMAEAYSEIGMKGERRRGKGHDGLYQGLSTATKDTYDALHMQALPPR

SEQ ID NO: 121 - DNA, 1386 bp, synthetic construct
  misc_feature 1..1386: note = Description of Artificial Sequence: Syntheticpolynucleotide
  source 1..1386: mol_type = other DNA
gagatcgtcatgacacagagtccagctaccctgagcgtgtcccctggagagagagccaccctgtcctgtagggctagtcagagtgtgtccagcctcctcacctggtatcaacagaagcctggtcaagctccccggctgcttatcttcggggccagcacgcgagccacaggcatcccggccagattctctggctctggcagtggcaccgggttcactctcacgatctcatccctgcagtcagaggatttcgctgtgtattactgtcagcagtacgatacatggcccttcaccttcggcccgggcacaaaagtagatttcaagcgcggcggcgggggtagtgggggcgggggatcaggaggagggggctcccaagtacagctggttgagagcggcggcggggtggttcagcccgggcgcagcctcaggctgagttgcgcagcatcaggattcacattcagttcttatggaatgcattgggtcagacaggctcccgggaagggccttgaatgggtggcagtcattagctacgacggaagcgataagtactatgtggactcagttaaagggagatttactatcagccgcgacaattccaaaaacagattgtatttgcagatgaactccctcagggcggaggacactgctgtatattactgcgcacgagagagatactccggccgagactattggggccaaggaacattggtaactgtgagctccgccgcagctattgaggtcatgtaccccccaccttatctcgataatgagaagagtaatgggactataattcacgtaaagggcaaacacctgtgcccttccccgctgtttccaggtccaagtaagccgttctgggtcctggttgtggtgggaggggtgctggcctgctattctctgttggttaccgtggcctttatcattttctgggtgagatccaaaagaagccgcctgctccatagcgattacatgaatatgactccacgccgccctggccccacaaggaaacactaccagccttacgcaccacctagagatttcgctgcctatcggagcagggtgaagttttccagatctgcagatgcaccagcgtatcagcagggccagaaccaactgtataacgagctcaacctgggacgcagggaagagtatgacgttttggacaagcgcagaggacgggaccctgagatgggtggcaaaccaagacgaaaaaacccccaggagggtctctataatgagctgcagaaggataagatggctgaagcctattctgaaataggcatgaaaggagagcggagaaggggaaaagggcacgacggtttgtaccagggactcagcactgctacgaaggatacttatgacgctctccacatgcaagccctgccacctagg

SEQ ID NO: 122 - protein, 462 aa, synthetic construct
  REGION 1..462: note = Description of Artificial Sequence: Syntheticpolypeptide
EIVMTQSPATLSVSPGERATLSCRASQSVSSLLTWYQQKPGQAPRLLIFGASTRATGIPARFSGSGSGTGFTLTISSLQSEDFAVYYCQQYDTWPFTFGPGTKVDFKRGGGGSGGGGSGGGGSQVQLVESGGGVVQPGRSLRLSCAASGFTFSSYGMHWVRQAPGKGLEWVAVISYDGSDKYYVDSVKGRFTISRDNSKNRLYLQMNSLRAEDTAVYYCARERYSGRDYWGQGTLVTVSSAAAIEVMYPPPYLDNEKSNGTIIHVKGKHLCPSPLFPGPSKPFWVLVVVGGVLACYSLLVTVAFIIFWVRSKRSRLLHSDYMNMTPRRPGPTRKHYQPYAPPRDFAAYRSRVKFSRSADAPAYQQGQNQLYNELNLGRREEYDVLDKRRGRDPEMGGKPRRKNPQEGLYNELQKDKMAEAYSEIGMKGERRRGKGHDGLYQGLSTATKDTYDALHMQALPPR

SEQ ID NO: 123 - DNA, 1533 bp, synthetic construct
  misc_feature 1..1533: note = Description of Artificial Sequence: Syntheticpolynucleotide
  source 1..1533: mol_type = other DNA
atggcactccccgtaactgctctgctgctgccgttggcattgctcctgcacgccgcacgcccggaaatagtgatgactcagtccccggccaccctcagcgtgtcccccggggagcgagcgaccctgtcatgcagggcttcccagagtgtcagctccctgctcacttggtatcagcaaaagccggggcaggctccccgcctcctcatcttcggggcatcaactagggccaccggcattcctgcaagattttccgggtctggcagcggcaccggcttcacccttaccattagctctctgcagtctgaggacttcgccgtttactattgtcagcagtatgatacttggccctttaccttcggtcccggaactaaggtggacttcaagcgcggggggggtggatctggaggtggtggctccgggggcggtggaagccaggtccagttggttgagagcggcggcggagtggtgcagcccgggaggtccttgcggctgagctgtgcagcctccggttttactttttctagctatggaatgcattgggtaagacaggctcccggaaaaggcctcgagtgggtggcggtcattagctatgatggatctgataaatactatgtggactcagttaaggggcgcttcacaatctcaagagacaatagcaaaaatagactgtacctgcagatgaatagtctgcgcgccgaggacactgccgtgtactactgcgcccgcgagagatacagcggacgggattactggggccagggtaccctcgtaacggtgtcctccgctgccgcccttagcaacagcattatgtacttttctcatttcgtgccagtctttctcccagcaaagcccaccactaccccggcccccaggccgcctactcctgcccccactatcgcgtctcagcctctctccttgcggcccgaggcctgccggccagccgcagggggcgccgtacatactcggggtttggatttcgcttgcgacatatatatttgggcccccctcgccggcacatgtggagtgctgctcctgagtctcgttataaccctctattgcaaccatagaaacagatccaaaagaagccgcctgctccatagcgattacatgaatatgactccacgccgccctggccccacaaggaaacactaccagccttacgcaccacctagagatttcgctgcctatcggagcagggtgaagttttccagatctgcagatgcaccagcgtatcagcagggccagaaccaactgtataacgagctcaacctgggacgcagggaagagtatgacgttttggacaagcgcagaggacgggaccctgagatgggtggcaaaccaagacgaaaaaacccccaggagggtctctataatgagctgcagaaggataagatggctgaagcctattctgaaataggcatgaaaggagagcggagaaggggaaaagggcacgacggtttgtaccagggactcagcactgctacgaaggatacttatgacgctctccacatgcaagccctgccacctaggtaa

SEQ ID NO: 124 - protein, 510 aa, synthetic construct
  REGION 1..510: note = Description of Artificial Sequence: Syntheticpolypeptide
MALPVTALLLPLALLLHAARPEIVMTQSPATLSVSPGERATLSCRASQSVSSLLTWYQQKPGQAPRLLIFGASTRATGIPARFSGSGSGTGFTLTISSLQSEDFAVYYCQQYDTWPFTFGPGTKVDFKRGGGGSGGGGSGGGGSQVQLVESGGGVVQPGRSLRLSCAASGFTFSSYGMHWVRQAPGKGLEWVAVISYDGSDKYYVDSVKGRFTISRDNSKNRLYLQMNSLRAEDTAVYYCARERYSGRDYWGQGTLVTVSSAAALSNSIMYFSHFVPVFLPAKPTTTPAPRPPTPAPTIASQPLSLRPEACRPAAGGAVHTRGLDFACDIYIWAPLAGTCGVLLLSLVITLYCNHRNRSKRSRLLHSDYMNMTPRRPGPTRKHYQPYAPPRDFAAYRSRVKFSRSADAPAYQQGQNQLYNELNLGRREEYDVLDKRRGRDPEMGGKPRRKNPQEGLYNELQKDKMAEAYSEIGMKGERRRGKGHDGLYQGLSTATKDTYDALHMQALPPR

SEQ ID NO: 125 - DNA, 1467 bp, synthetic construct
  misc_feature 1..1467: note = Description of Artificial Sequence: Syntheticpolynucleotide
  source 1..1467: mol_type = other DNA
gaaatagtgatgactcagtccccggccaccctcagcgtgtcccccggggagcgagcgaccctgtcatgcagggcttcccagagtgtcagctccctgctcacttggtatcagcaaaagccggggcaggctccccgcctcctcatcttcggggcatcaactagggccaccggcattcctgcaagattttccgggtctggcagcggcaccggcttcacccttaccattagctctctgcagtctgaggacttcgccgtttactattgtcagcagtatgatacttggccctttaccttcggtcccggaactaaggtggacttcaagcgcggggggggtggatctggaggtggtggctccgggggcggtggaagccaggtccagttggttgagagcggcggcggagtggtgcagcccgggaggtccttgcggctgagctgtgcagcctccggttttactttttctagctatggaatgcattgggtaagacaggctcccggaaaaggcctcgagtgggtggcggtcattagctatgatggatctgataaatactatgtggactcagttaaggggcgcttcacaatctcaagagacaatagcaaaaatagactgtacctgcagatgaatagtctgcgcgccgaggacactgccgtgtactactgcgcccgcgagagatacagcggacgggattactggggccagggtaccctcgtaacggtgtcctccgctgccgcccttagcaacagcattatgtacttttctcatttcgtgccagtctttctcccagcaaagcccaccactaccccggcccccaggccgcctactcctgcccccactatcgcgtctcagcctctctccttgcggcccgaggcctgccggccagccgcagggggcgccgtacatactcggggtttggatttcgcttgcgacatatatatttgggcccccctcgccggcacatgtggagtgctgctcctgagtctcgttataaccctctattgcaaccatagaaacagatccaaaagaagccgcctgctccatagcgattacatgaatatgactccacgccgccctggccccacaaggaaacactaccagccttacgcaccacctagagatttcgctgcctatcggagcagggtgaagttttccagatctgcagatgcaccagcgtatcagcagggccagaaccaactgtataacgagctcaacctgggacgcagggaagagtatgacgttttggacaagcgcagaggacgggaccctgagatgggtggcaaaccaagacgaaaaaacccccaggagggtctctataatgagctgcagaaggataagatggctgaagcctattctgaaataggcatgaaaggagagcggagaaggggaaaagggcacgacggtttgtaccagggactcagcactgctacgaaggatacttatgacgctctccacatgcaagccctgccacctagg

SEQ ID NO: 126 - protein, 489 aa, synthetic construct
  REGION 1..489: note = Description of Artificial Sequence: Syntheticpolypeptide
EIVMTQSPATLSVSPGERATLSCRASQSVSSLLTWYQQKPGQAPRLLIFGASTRATGIPARFSGSGSGTGFTLTISSLQSEDFAVYYCQQYDTWPFTFGPGTKVDFKRGGGGSGGGGSGGGGSQVQLVESGGGVVQPGRSLRLSCAASGFTFSSYGMHWVRQAPGKGLEWVAVISYDGSDKYYVDSVKGRFTISRDNSKNRLYLQMNSLRAEDTAVYYCARERYSGRDYWGQGTLVTVSSAAALSNSIMYFSHFVPVFLPAKPTTTPAPRPPTPAPTIASQPLSLRPEACRPAAGGAVHTRGLDFACDIYIWAPLAGTCGVLLLSLVITLYCNHRNRSKRSRLLHSDYMNMTPRRPGPTRKHYQPYAPPRDFAAYRSRVKFSRSADAPAYQQGQNQLYNELNLGRREEYDVLDKRRGRDPEMGGKPRRKNPQEGLYNELQKDKMAEAYSEIGMKGERRRGKGHDGLYQGLSTATKDTYDALHMQALPPR

SEQ ID NO: 127 - DNA, 63 bp, Homo sapiens
  source 1..63: mol_type = other DNA
atggcactccccgtaactgctctgctgctgccgttggcattgctcctgcacgccgcacgcccg

SEQ ID NO: 128 - protein, 21 aa, Homo sapiens
MALPVTALLLPLALLLHAARP

SEQ ID NO: 129 - DNA, 45 bp, synthetic construct
  misc_feature 1..45: note = Description of Artificial Sequence: Syntheticoligonucleotide
  source 1..45: mol_type = other DNA
ggcggtggaggctccggaggggggggctctggcggagggggctcc

SEQ ID NO: 130 - protein, 15 aa, synthetic construct
  REGION 1..15: note = Description of Artificial Sequence: Syntheticpeptide
GGGGSGGGGSGGGGS

SEQ ID NO: 131 - DNA, 54 bp, synthetic construct
  misc_feature 1..54: note = Description of Artificial Sequence: Syntheticoligonucleotide
  source 1..54: mol_type = other DNA
gggtctacatccggctccgggaagcccggaagtggcgaaggtagtacaaagggg

SEQ ID NO: 132 - protein, 18 aa, synthetic construct
  REGION 1..18: note = Description of Artificial Sequence: Syntheticpeptide
GSTSGSGKPGSGEGSTKG

SEQ ID NO: 133 - protein, 152 aa, Homo sapiens
MLRLLLALNLFPSIQVTGNKILVKQSPMLVAYDNAVNLSCKYSYNLFSREFRASLHKGLDSAVEVCVVYGNYSQQLQVYSKTGFNCDGKLGNESVTFYLQNLYVNQTDIYFCKIEVMYPPPYLDNEKSNGTIIHVKGKHLCPSPLFPGPSKP

SEQ ID NO: 134-135 - skipped (2 entries)

SEQ ID NO: 136 - protein, 14 aa, synthetic construct
  REGION 1..14: note = Description of Artificial Sequence: Syntheticpeptide
  MOD_RES 1: note = Glu or Leu
  MOD_RES 2: note = Arg, Ser or Val
  MOD_RES 3: note = Arg or Tyr
  MOD_RES 4: note = Cys, Gly or Ser
  MOD_RES 5: note = Gly, Ile or absent
  MOD_RES 6..8: note = May or may not be present
  MOD_RES 9: note = Trp, Tyr or absent
  MOD_RES 10: note = Pro, Ser or absent
  MOD_RES 11: note = Gly, Tyr or absent
  MOD_RES 12: note = Phe or Arg
XXXXXGDCXXXXDY

SEQ ID NO: 137 - protein, 11 aa, synthetic construct
  REGION 1..11: note = Description of Artificial Sequence: Syntheticpeptide
  MOD_RES 1: note = Gln or Arg
  MOD_RES 5: note = Asp or Ser
  MOD_RES 6: note = Ile or Val
  MOD_RES 7..8: note = Asn or Ser
  MOD_RES 9: note = Phe, Leu or Tyr
  MOD_RES 11: note = Asn or Thr
XASQXXXXXLX

SEQ ID NO: 138 - skipped

SEQ ID NO: 139 - protein, 9 aa, synthetic construct
  REGION 1..9: note = Description of Artificial Sequence: Syntheticpeptide
  MOD_RES 3: note = Ser or Tyr
  MOD_RES 4: note = Asp, Gly or Tyr
  MOD_RES 5: note = Asn, Ser or Thr
  MOD_RES 6: note = Leu, Thr or Tyr
  MOD_RES 8: note = Phe or Ile
QQXXXXPXT

SEQ ID NO: 140 - protein, 265 aa, Homo sapiens
MSEEVTYADLQFQNSSEMEKIPEIGKFGEKAPPAPSHVWRPAALFLTLLCLLLLIGLGVLASMFHVTLKIEMKKMNKLQNISEELQRNISLQLMSNMNISNKIRNLSTTLQTIATKLCRELYSKEQEHKCKPCPRRWIWHKDSCYFLSDDVQTWQESKMACAAQNASLLKINNKNALEFIKSQSRSYDYWLGLSPEEDSTRGMRVDNIINSSAWVIRNAPDLNNMYCGYINRLYVQYYHCTYKKRMICEKMANPVQLGSTYFREA

SEQ ID NO: 141 - DNA, 126 bp, Homo sapiens
  source 1..126: mol_type = other DNA
aagcgcggcaggaagaagctcctctacatttttaagcagccttttatgaggcccgtacagacaacacaggaggaagatggctgtagctgcagatttcccgaggaggaggaaggtgggtgcgagctg

SEQ ID NO: 142 - protein, 42 aa, Homo sapiens
KRGRKKLLYIFKQPFMRPVQTTQEEDGCSCRFPEEEEGGCEL

SEQ ID NO: 143 - protein, 37 aa, Homo sapiens
RRDQRLPPDAHKPPGGGSFRTPIQEEQADAHSTLAKI

SEQ ID NO: 144 - protein, 21 aa, synthetic construct
  REGION 1..21: note = Description of Artificial Sequence: Syntheticpeptide
MALPVTALLLPLALLLHAARP

SEQ ID NO: 145 - protein, 20 aa, synthetic construct
  REGION 1..20: note = Description of Artificial Sequence: Syntheticpeptide
GGGGSGGGGSGGGGSGGGGS

SEQ ID NO: 146 - protein, 112 aa, Homo sapiens
RVKFSRSADAPAYKQGQNQLYNELNLGRREEYDVLDKRRGRDPEMGGKPRRKNPQEGLYNELQKDKMAEAYSEIGMKGERRRGKGHDGLYQGLSTATKDTYDALHMQALPPR

SEQ ID NO: 147 - DNA, 6762 bp, synthetic construct
  source 1..6762: mol_type = other DNA
ctgacgcgccctgtagcggcgcattaagcgcggcgggtgtggtggttacgcgcagcgtgaccgctacacttgccagcgccctagcgcccgctcctttcgctttcttcccttcctttctcgccacgttcgccggctttccccgtcaagctctaaatcgggggctccctttagggttccgatttagtgctttacggcacctcgaccccaaaaaacttgattagggtgatggttcacgtagtgggccatcgccctgatagacggtttttcgccctttgacgttggagtccacgttctttaatagtggactcttgttccaaactggaacaacactcaaccctatctcggtctattcttttgatttataagggattttgccgatttcggcctattggttaaaaaatgagctgatttaacaaaaatttaacgcgaattttaacaaaatattaacgcttacaatttgccattcgccattcaggctgcgcaactgttgggaagggcgatcggtgcgggcctcttcgctattacgccagctggcgaaagggggatgtgctgcaaggcgattaagttgggtaacgccagggttttcccagtcacgacgttgtaaaacgacggccagtgaattgtaatacgactcactatagggcgacccggggatggcgcgccagtaatcaattacggggtcattagttcatagcccatatatggagttccgcgttacataacttacggtaaatggcccgcctggctgaccgcccaacgacccccgcccattgacgtcaataatgacgtatgttcccatagtaacgccaatagggactttccattgacgtcaatgggtggagtatttacggtaaactgcccacttggcagtacatcaagtgtatcatatgccaagtacgccccctattgacgtcaatgacggtaaatggcccgcctggcattatgcccagtacatgaccttatgggactttcctacttggcagtacatctacgtattagtcatcgctattaccatgctgatgcggttttggcagtacatcaatgggcgtggatagcggtttgactcacggggatttccaagtctccaccccattgacgtcaatgggagtttgttttggcaccaaaatcaacgggactttccaaaatgtcgtaacaactccgccccattgacgcaaatgggcggtaggcgtgtacggtgggaggtctatataagcagagctggtttagtgaaccggggtctctctggttagaccagatctgagcctgggagctctctggctaactagggaacccactgcttaagcctcaataaagcttgccttgagtgcttcaagtagtgtgtgcccgtctgttgtgtgactctggtaactagagatccctcagacccttttagtcagtgtggaaaatctctagcagtggcgcccgaacagggacttgaaagcgaaagggaaaccagaggagctctctcgacgcaggactcggcttgctgaagcgcgcacggcaagaggcgaggggcggcgactggtgagtacgccaaaaattttgactagcggaggctagaaggagagagatgggtgcgagagcgtcagtattaagcgggggagaattagatcgcgatgggaaaaaattcggttaaggccagggggaaagaaaaaatataaattaaaacatatagtatgggcaagcagggagctagaacgattcgcagttaatcctggcctgttagaaacatcagaaggctgtagacaaatactgggacagctacaaccatcccttcagacaggatcagaagaacttagatcattatataatacagtagcaaccctctattgtgtgcatcaaaggatagagataaaagacaccaaggaagctttagacaagatagaggaagagcaaaacaaaagtaagaccaccgcacagcaagccgccgctgatcttcagacctggaggaggagatatgagggacaattggagaagtgaattatataaatataaagtagtaaaaattgaaccattaggagtagcacccaccaaggcaaagagaagagtggtgcagagagaaaaaagagcagtgggaataggagctttgttccttgggttcttgggagcagcaggaagcactatgggcgcagcgtcaatgacgctgacggtacaggccagacaattattgtctggtatagtgcagcagcagaacaatttgctgagggctattgaggcgcaacagcatctgttgcaactcacagtctggggcatcaagcagctccaggcaagaatcctggctgtggaaagatacctaaaggatcaacagctcctggggatttggggttgctctggaaaactcatttgcaccactgctgtgccttggaatgctagttggagtaataaatctctggaacagatttggaatcacacgacctggatggagtgggacagagaaattaacaattacacaagcttaatacactccttaattgaagaatcgcaaaaccagcaagaaaagaatgaacaagaattattggaattagataaatgggcaagtttgtggaattggtttaacataacaaattggctgtggtatataaaattattcataatgatagtaggaggcttggtaggtttaagaatagtttttgctgtactttctatagtgaatagagttaggcagggatattcaccattatcgtttcagacccacctcccaaccccgaggggacccgacaggcccgaaggaatagaagaagaaggtggagagagagacagagacagatccattcgattagtgaacggatctcgacggtatcggttaacttttaaaagaaaaggggggattggggggtacagtgcaggggaaagaatagtagacataatagcaacagacatacaaactaaagaattacaaaaacaaattacaaaattcaaaattttatcgcgatcgcggaatgaaagaccccacctgtaggtttggcaagctagcttaagtaacgccattttgcaaggcatggaaaatacataactgagaatagagaagttcagatcaaggttaggaacagagagacagcagaatatgggccaaacaggatatctgtggtaagcagttcctgccccggctcagggccaagaacagatggtccccagatgcggtcccgccctcagcagtttctagagaaccatcagatgtttccagggtgccccaaggacctgaaaatgaccctgtgccttatttgaactaaccaatcagttcgcttctcgcttctgttcgcgcgcttctgctccccgagctcaataaaagagcccacaacccctcactcggcgcgccagtccttcgaagtagatctttgtcgatcctaccatccactcgacacacccgccagcggccgctgccaagcttccgagctctcgaattaattcacggtacccaccatggcctagggagactagtcgaatcgatatcaacctctggattacaaaatttgtgaaagattgactggtattcttaactatgttgctccttttacgctatgtggatacgctgctttaatgcctttgtatcatgctattgcttcccgtatggctttcattttctcctccttgtataaatcctggttgctgtctctttatgaggagttgtggcccgttgtcaggcaacgtggcgtggtgtgcactgtgtttgctgacgcaacccccactggttggggcattgccaccacctgtcagctcctttccgggactttcgctttccccctccctattgccacggcggaactcatcgccgcctgccttgcccgctgctggacaggggctcggctgttgggcactgacaattccgtggtgttgtcggggaagctgacgtccttttcatggctgctcgcctgtgttgccacctggattctgcgcgggacgtccttctgctacgtcccttcggccctcaatccagcggaccttccttcccgcggcctgctgccggctctgcggcctcttccgcgtcttcgccttcgccctcagacgagtcggatctccctttgggccgcctccccgcctggttaattaaagtacctttaagaccaatgacttacaaggcagctgtagatcttagccactttttaaaagaaaaggggggactggaagggcgaattcactcccaacgaagacaagatctgctttttgcttgtactgggtctctctggttagaccagatctgagcctgggagctctctggctaactagggaacccactgcttaagcctcaataaagcttgccttgagtgcttcaagtagtgtgtgcccgtctgttgtgtgactctggtaactagagatccctcagacccttttagtcagtgtggaaaatctctagcaggcatgccagacatgataagatacattgatgagtttggacaaaccacaactagaatgcagtgaaaaaaatgctttatttgtgaaatttgtgatgctattgctttatttgtaaccattataagctgcaataaacaagttaacaacaacaattgcattcattttatgtttcaggttcagggggaggtgtgggaggttttttggcgcgccatcgtcgaggttccctttagtgagggttaattgcgagcttggcgtaatcatggtcatagctgtttcctgtgtgaaattgttatccgctcacaattccacacaacatacgagccggaagcataaagtgtaaagcctggggtgcctaatgagtgagctaactcacattaattgcgttgcgctcactgcccgctttccagtcgggaaacctgtcgtgccagctgcattaatgaatcggccaacgcgcggggagaggcggtttgcgtattgggcgctcttccgcttcctcgctcactgactcgctgcgctcggtcgttcggctgcggcgagcggtatcagctcactcaaaggcggtaatacggttatccacagaatcaggggataacgcaggaaagaacatgtgagcaaaaggccagcaaaaggccaggaaccgtaaaaaggccgcgttgctggcgtttttccataggctccgcccccctgacgagcatcacaaaaatcgacgctcaagtcagaggtggcgaaacccgacaggactataaagataccaggcgtttccccctggaagctccctcgtgcgctctcctgttccgaccctgccgcttaccggatacctgtccgcctttctcccttcgggaagcgtggcgctttctcatagctcacgctgtaggtatctcagttcggtgtaggtcgttcgctccaagctgggctgtgtgcacgaaccccccgttcagcccgaccgctgcgccttatccggtaactatcgtcttgagtccaacccggtaagacacgacttatcgccactggcagcagccactggtaacaggattagcagagcgaggtatgtaggcggtgctacagagttcttgaagtggtggcctaactacggctacactagaagaacagtatttggtatctgcgctctgctgaagccagttaccttcggaaaaagagttggtagctcttgatccggcaaacaaaccaccgctggtagcggtggtttttttgtttgcaagcagcagattacgcgcagaaaaaaaggatctcaagaagatcctttgatcttttctacggggtctgacgctcagtggaacgaaaactcacgttaagggattttggtcatgagattatcaaaaaggatcttcacctagatccttttaaattaaaaatgaagttttaaatcaatctaaagtatatatgagtaaacttggtctgacagttaccaatgcttaatcagtgaggcacctatctcagcgatctgtctatttcgttcatccatagttgcctgactccccgtcgtgtagataactacgatacgggagggcttaccatctggccccagtgctgcaatgataccgcgagacccacgctcaccggctccagatttatcagcaataaaccagccagccggaagggccgagcgcagaagtggtcctgcaactttatccgcctccatccagtctattaattgttgccgggaagctagagtaagtagttcgccagttaatagtttgcgcaacgttgttgccattgctacaggcatcgtggtgtcacgctcgtcgtttggtatggcttcattcagctccggttcccaacgatcaaggcgagttacatgatcccccatgttgtgcaaaaaagcggttagctccttcggtcctccgatcgttgtcagaagtaagttggccgcagtgttatcactcatggttatggcagcactgcataattctcttactgtcatgccatccgtaagatgcttttctgtgactggtgagtactcaaccaagtcattctgagaatagtgtatgcggcgaccgagttgctcttgcccggcgtcaatacgggataataccgcgccacatagcagaactttaaaagtgctcatcattggaaaacgttcttcggggcgaaaactctcaaggatcttaccgctgttgagatccagttcgatgtaacccactcgtgcacccaactgatcttcagcatcttttactttcaccagcgtttctgggtgagcaaaaacaggaaggcaaaatgccgcaaaaaagggaataagggcgacacggaaatgttgaatactcatactcttcctttttcaatattattgaagcatttatcagggttattgtctcatgagcggatacatatttgaatgtatttagaaaaataaacaaataggggttccgcgcacatttccccgaaaagtgccac